European Patent Specification EP 2 954 049 B1, published May 17, 2023. Title: ATTENUATION OF HUMAN RESPIRATORY SYNCYTIAL VIRUS BY GENOME SCALE CODON-PAIR DEOPTIMIZATION. Applicant: THE UNITED STATES OF AMERICA, AS REPRESENTED BY THE SECRETARY, DEPARTMENT OF HEALTH AND HUMAN SERVICES. The sequence listing filed with the application follows.

SEQUENCE LISTING (5 sequences)

SEQ ID NO: 1 - DNA, 15111 bp, Human respiratory syncytial virus
acgggaaaaaatgcgtacaacaaacttgcataaaccaaaaaaatggggcaaataagaatttgataagtaccacttaaatttaactcccttggttagagatgggcagcaattcattgagtatgataaaagttagattacaaaatttgtttgacaatgatgaagtagcattgttaaaaataacatgctatactgataaattaatacatttaactaatgctttggctaaggcagtgatacatacaatcaaattgaatggcattgtgtttgtgcatgttattacaagtagtgatatttgccctaataataatattgtagtaaaatccaatttcacaacaatgccagtactacaaaatggaggttatatatgggaaatgatggaattaacacattgctctcaacctaatggtctactagatgacaattgtgaaattaaattctccaaaaaactaagtgattcaacaatgaccaattatatgaatcaattatctgaattacttggatttgatcttaatccataaattataattaatatcaactagcaaatcaatgtcactaacaccattagttaatataaaacttaacagaagacaaaaatggggcaaataaatcaattcagccaacccaaccatggacacaacccacaatgataatacaccacaaagactgatgatcacagacatgagaccgttgtcacttgagaccataataacatcactaaccagagacatcataacacacaaatttatatacttgataaatcatgaatgcatagtgagaaaacttgatgaaagacaggccacatttacattcctggtcaactatgaaatgaaactattacacaaagtaggaagcactaaatataaaaaatatactgaatacaacacaaaatatggcactttccctatgccaatattcatcaatcatgatgggttcttagaatgcattggcattaagcctacaaagcatactcccataatatacaagtatgatctcaatccataaatttcaacacaatattcacacaatctaaaacaacaactctatgcataactatactccatagtccagatggagcctgaaaattatagtaatttaaaacttaaggagagatataagatagaagatggggcaaatacaaccatggctcttagcaaagtcaagttgaatgatacactcaacaaagatcaacttctgtcatccagcaaatacaccatccaacggagcacaggagatagtattgatactcctaattatgatgtgcagaaacacatcaataagttatgtggcatgttattaatcacagaagatgctaatcataaattcactgggttaataggtatgttatatgcgatgtctaggttaggaagagaagacaccataaaaatactcagagatgcgggatatcatgtaaaagcaaatggagtagatgtaacaacacatcgtcaagacattaatggaaaagaaatgaaatttgaagtgttaacattggcaagcttaacaactgaaattcaaatcaacattgagatagaatctagaaaatcctacaaaaaaatgctaaaagaaatgggagaggtagctccagaatacaggcatgactctcctgattgtgggatgataatattatgtatagcagcattagtaataactaaattagcagcaggggacagatctggtcttacagccgtgattaggagagctaataatgtcctaaaaaatgaaatgaaacgttacaaaggcttactacccaaggacatagccaacagcttctatgaagtgtttgaaaaacatccccactttatagatgtttttgttcattttggtatagcacaatcttctaccagaggtggcagtagagttgaagggatttttgcaggattgtttatgaatgcctatggtgcagggcaagtgatgttacggtggggagtcttagcaaaatcggttaaaaatattatgttaggacatgctagtgtgcaagcagaaatggaacaagttgttgaggtttatgaatatgcccaaaaattgggtggtgaagcaggattctaccatatattgaacaacccaaaagcatcattattatctttgactcaatttcctcacttctccagtgtagtattaggcaatgctgctggcctaggcataatgggagagtacagaggtacaccgaggaatcaagatctatatgatgcagcaaaggcatatgctgaacaactcaaagaaaatggtgtgattaactacagtgtactagacttgacagcagaagaactagaggctatcaaacatcagcttaatccaaaagataatgatgtagagctttgagttaataaaaaatggggcaaataaatcatcatggaaaagtttgctcctgaattccatggagaagatgcaaacaacagggctactaaattcctagaatcaataaagggcaaattcacatcacccaaagatcccaagaaaaaagatagtatcatatctgtcaactcaatagatatagaagtaaccaaagaaagccctataacatcaaattcaactattatcaacccaacaaatgagacagatgatactgcagggaacaagcccaattatcaaagaaaacctctagtaagtttcaaagaagaccctacaccaagtgataatcccttttctaaactatacaaagaaaccatagaaacatttgataacaatgaagaagaatccagctattcatacgaagaaataaatgatcagacaaacgataatataacagcaagattagataggattgatgaaaaattaagtgaaatactaggaatgcttcacacattagtagtggcaagtgcaggacctacatctgctcgggatggtataagagatgccatggttggtttaagagaagaaatgatagaaaaaatcagaactgaagcattaatgaccaatgacagattagaagctatggcaagactcaggaatgaggaaagtgaaaagatggcaaaagacacatcagatgaagtgtctctcaatccaacatcagagaaattgaacaacctattggaagggaatgatagtgacaatgatctatcacttgaagatttctgattagttaccaatcttcacatcaacacacaataccaacagaagaccaacaaactaaccaacccaatcatccaaccaaacatccatccgccaatcagccaaacagccaacaaaacaaccagccaatccaaaactaaccacccggaaaaaatctataatatagttacaaaaaaaggaaagggtggggcaaatatggaaacatacgtgaacaagcttcacgaaggctccacatacacagctgctgttcaatacaatgtcttagaaaaagacgatgaccctgcatcacttacaatatgggtgcccatgttccaatcatctatgccagcagatttacttataaaagaactagctaatgtcaacatactagtgaaacaaatatccacacccaagggaccttcactaagagtcatgataaactcaagaagtgcagtgctagcacaaatgcccagcaaatttaccatatgcgctaatgtgtccttggatgaaagaagcaaactagcatatgatgtaaccacaccctgtgaaatcaaggcatgtagtctaacatgcctaaaatcaaaaaatatgttgactacagttaaagatctcactatgaagacactcaaccctacacatgatattattgctttatgtgaatttgaaaacatagtaacatcaaaaaaagtcataataccaacatacctaagatccatcagtgtcagaaataaagatctgaacacacttgaaaatataacaaccactgaattcaaaaatgctatcacaaatgcaaaaatcatcccttactcaggattactattagtcatcacagtgactgacaacaaaggagcattcaaatacataaagccacaaagtcaattcatagtagatcttggagcttacctagaaaaagaaagtatatattatgttaccacaaattggaagcacacagctacacgatttgcaatcaaacccatggaagattaacctttttcctctacatcagtgtgttaattcatacaaactttctacctacattcttcacttcaccatcacaatcacaaacactctgtggttcaaccaatcaaacaaaacttatctgaagtcccagatcatcccaagtcattgtttatcagatctagtactcaaataagttaataaaaaatatacacatggggcaaataatcattggaggaaatccaactaatcacaatatctgttaacatagacaagtccacacaccatacagaatcaaccaatggaaaatacatccataacaatagaattctcaagcaaattctggccttactttacactaatacacatgatcacaacaataatctctttgctaatcataatctccatcatgattgcaatactaaacaaactttgtgaatataacgtattccataacaaaacctttgagttaccaagagctcgagttaatacttgataaagtagttaattaaaaatagtcataacaatgaactaggatatcaagactaacaataacattggggcaaatgcaaacatgtccaaaaacaaggaccaacgcaccgctaagacattagaaaggacctgggacactctcaatcatttattattcatatcatcgtgcttatataagttaaatcttaaatctgtagcacaaatcacattatccattctggcaatgataatctcaacttcacttataattgcagccatcatattcatagcctcggcaaaccacaaagtcacaccaacaactgcaatcatacaagatgcaacaagccagatcaagaacacaaccccaacatacctcacccagaatcctcagcttggaatcagtccctctaatccgtctgaaattacatcacaaatcaccaccatactagcttcaacaacaccaggagtcaagtcaaccctgcaatccacaacagtcaagaccaaaaacacaacaacaactcaaacacaacccagcaagcccaccacaaaacaacgccaaaacaaaccaccaagcaaacccaataatgattttcactttgaagtgttcaactttgtaccctgcagcatatgcagcaacaatccaacctgctgggctatctgcaaaagaataccaaacaaaaaaccaggaaagaaaaccactaccaagcccacaaaaaaaccaaccctcaagacaaccaaaaaagatcccaaacctcaaaccactaaatcaaaggaagtacccaccaccaagcccacagaagagccaaccatcaacaccaccaaaacaaacatcataactacactactcacctccaacaccacaggaaatccagaactcacaagtcaaatggaaaccttccactcaacttcctccgaaggcaatccaagcccttctcaagtctctacaacatccgagtacccatcacaaccttcatctccacccaacacaccacgccagtagttacttaaaaacatattatcacaaaaggccttgaccaacttaaacagaatcaaaataaactctggggcaaataacaatggagttgctaatcctcaaagcaaatgcaattaccacaatcctcactgcagtcacattttgttttgcttctggtcaaaacatcactgaagaattttatcaatcaacatgcagtgcagttagcaaaggctatcttagtgctctgagaactggttggtataccagtgttataactatagaattaagtaatatcaagaaaaataagtgtaatggaacagatgctaaggtaaaattgataaaacaagaattagataaatataaaaatgctgtaacagaattgcagttgctcatgcaaagcacacaagcaacaaacaatcgagccagaagagaactaccaaggtttatgaattatacactcaacaatgccaaaaaaaccaatgtaacattaagcaagaaaaggaaaagaagatttcttggttttttgttaggtgttggatctgcaatcgccagtggcgttgctgtatctaaggtcctgcacctagaaggggaagtgaacaagatcaaaagtgctctactatccacaaacaaggctgtagtcagcttatcaaatggagttagtgttttaaccagcaaagtgttagacctcaaaaactatatagataaacaattgttacctattgtgaacaagcaaagctgcagcatatcaaatatagaaactgtgatagagttccaacaaaagaacaacagactactagagattaccagggaatttagtgttaatgcaggcgtaactacacctgtaagcacttacatgttaactaatagtgaattattgtcattaatcaatgatatgcctataacaaatgatcagaaaaagttaatgtccaacaatgttcaaatagttagacagcaaagttactctatcatgtccataataaaagaggaagtcttagcatatgtagtacaattaccactatatggtgttatagatacaccctgttggaaactacacacatcccctctatgtacaaccaacacaaaagaagggtccaacatctgtttaacaagaactgacagaggatggtactgtgacaatgcaggatcagtatctttcttcccacaagctgaaacatgtaaagttcaatcaaatcgagtattttgtgacacaatgaacagtttaacattaccaagtgaagtaaatctctgcaatgttgacatattcaaccccaaatatgattgtaaaattatgacttcaaaaacagatgtaagcagctccgttatcacatctctaggagccattgtgtcatgctatggcaaaactaaatgtacagcatccaataaaaatcgtggaatcataaagacattttctaacgggtgcgattatgtatcaaataaaggggtggacactgtgtctgtaggtaacacattatattatgtaaataagcaagaaggtaaaagtctctatgtaaaaggtgaaccaataataaatttctatgacccattagtattcccctctgatgaatttgatgcatcaatatctcaagtcaacgagaagattaaccagagcctagcatttattcgtaaatccgatgaattattacataatgtaaatgctggtaaatccaccacaaatatcatgataactactataattatagtgattatagtaatattgttatcattaattgctgttggactgctcttatactgtaaggccagaagcacaccagtcacactaagcaaagatcaactgagtggtataaataatattgcatttagtaactaaataaaaatagcacctaatcatgttcttacaatggtttactatctgctcatagacaacccatctgtcattggattttcttaaaatctgaacttcatcgaaactctcatctataaaccatctcacttacactatttaagtagattcctagtttatagttatataaaacacaattgcatgccagattaacttaccatctgtaaaaatgaaaactggggcaaatatgtcacgaaggaatccttgcaaatttgaaattcgaggtcattgcttaaatggtaagaggtgtcattttagtcataattattttgaatggccaccccatgcactgcttgtaagacaaaactttatgttaaacagaatacttaagtctatggataaaagtatagataccttatcagaaataagtggagctgcagagttggacagaacagaagagtatgctcttggtgtagttggagtgctagagagttatataggatcaataaacaatataactaaacaatcagcatgtgttgccatgagcaaactcctcactgaactcaatagtgatgatatcaaaaagctgagggacaatgaagagctaaattcacccaagataagagtgtacaatactgtcatatcatatattgaaagcaacaggaaaaacaataaacaaactatccatctgttaaaaagattgccagcagacgtattgaagaaaaccatcaaaaacacattggatatccataagagcataaccatcaacaacccaaaagaatcaactgttagtgatacaaatgaccatgccaaaaataatgatactacctgacaaatatccttgtagtataacttccatactaataacaagtagatgtagagttactatgtataatcaaaagaacacactatatttcaatcaaaacaacccaaataaccatatgtactcaccgaatcaaacattcaatgaaatccattggacctctcaagaattgattgacacaattcaaaattttctacaacatctaggtattattgaggatatatatacaatatatatattagtgtcataacactcaattctaacactcaccacatcgttacattattaattcaaacaattcaagttgtgggacaaaatggatcccattattaatggaaattctgctaatgtttatctaaccgatagttatttaaaaggtgttatctctttctcagagtgtaatgctttaggaagttacatattcaatggtccttatctcaaaaatgattataccaacttaattagtagacaaaatccattaatagaacacatgaatctaaagaaactaaatataacacagtccttaatatctaagtatcataaaggtgaaataaaattagaagaacctacttattttcagtcattacttatgacatacaagagtatgacctcgtcagaacagattgctaccactaatttacttaaaaagataataagaagagctatagaaataagtgatgtcaaagtctatgctatattgaataaactagggcttaaagaaaaggacaagattaaatccaacaatggacaagatgaagacaactcagttattacgaccataatcaaagatgatatactttcagctgttaaagataatcaatctcatcttaaagcagacaaaaatcactctacaaaacaaaaagacacaatcaaaacaacactcttgaagaaattgatgtgttcaatgcaacatcctccatcatggttaatacattggtttaacttatacacaaaattaaacaacatattaacacagtatcgatcaaatgaggtaaaaaaccatgggtttacattgatagataatcaaactcttagtggatttcaatttattttgaaccaatatggttgtatagtttatcataaggaactcaaaagaattactgtgacaacctataatcaattcttgacatggaaagatattagccttagtagattaaatgtttgtttaattacatggattagtaactgcttgaacacattaaataaaagcttaggcttaagatgcggattcaataatgttatcttgacacaactattcctttatggagattgtatactaaagctatttcacaatgaggggttctacataataaaagaggtagagggatttattatgtctctaattttaaatataacagaagaagatcaattcagaaaacgattttataatagtatgctcaacaacatcacagatgctgctaataaagctcagaaaaatctgctatcaagagtatgtcatacattattagataagacagtgtccgataatataataaatggcagatggataattctattaagtaagttccttaaattaattaagcttgcaggtgacaataaccttaacaatctgagtgaactatattttttgttcagaatatttggacacccaatggtagatgaaagacaagccatggatgctgttaaaattaattgcaatgagaccaaattttacttgttaagcagtctgagtatgttaagaggtgcctttatatatagaattataaaagggtttgtaaataattacaacagatggcctactttaagaaatgctattgttttacccttaagatggttaacttactataaactaaacacttatccttctttgttggaacttacagaaagagatttgattgtgttatcaggactacgtttctatcgtgagtttcggttgcctaaaaaagtggatcttgaaatgattataaatgataaagctatatcacctcctaaaaatttgatatggactagtttccctagaaattacatgccatcacacatacaaaactatatagaacatgaaaaattaaaattttccgagagtgataaatcaagaagagtattagagtattatttaagagataacaaattcaatgaatgtgatttatacaactgtgtagttaatcaaagttatctcaacaaccctaatcatgtggtatcattgacaggcaaagaaagagaactcagtgtaggtagaatgtttgcaatgcaaccgggaatgttcagacaggttcaaatattggcagagaaaatgatagctgaaaacattttacaattctttcctgaaagtcttacaagatatggtgatctagaactacaaaaaatattagaactgaaagcaggaataagtaacaaatcaaatcgctacaatgataattacaacaattacattagtaagtgctctatcatcacagatctcagcaaattcaatcaagcatttcgatatgaaacgtcatgtatttgtagtgatgtgctggatgaactgcatggtgtacaatctctattttcctggttacatttaactattcctcatgtcacaataatatgcacatataggcatgcacccccctatataggagatcatattgtagatcttaacaatgtagatgaacaaagtggattatatagatatcacatgggtggcatcgaagggtggtgtcaaaaactatggaccatagaagctatatcactattggatctaatatctctcaaagggaaattctcaattactgctttaattaatggtgacaatcaatcaatagatataagcaaaccaatcagactcatggaaggtcaaactcatgctcaagcagattatttgctagcattaaatagccttaaattactgtataaagagtatgcaggcataggccacaaattaaaaggaactgagacttatatatcacgagatatgcaatttatgagtaaaacaattcaacataacggtgtatattacccagctagtataaagaaagtcctaagagtgggaccgtggataaacactatacttgatgatttcaaagtgagtctagaatctataggtagtttgacacaagaattagaatatagaggtgaaagtctattatgcagtttaatatttagaaatgtatggttatataatcagattgctctacaattaaaaaatcatgcattatgtaacaataaactatatttggacatattaaaggttctgaaacacttaaaaaccttttttaatcttgataatattgatacagcattaacattgtatatgaatttacccatgttatttggtggtggtgatcccaacttgttatatcgaagtttctatagaagaactcctgacttcctcacagaggctatagttcactctgtgttcatacttagttattatacaaaccatgacttaaaagataaacttcaagatctgtcagatgatagattgaataagttcttaacatgcataatcacgtttgacaaaaaccctaatgctgaattcgtaacattgatgagagatcctcaagctttagggtctgagagacaagctaaaattactagcgaaatcaatagactggcagttacagaggttttgagtacagctccaaacaaaatattctccaaaagtgcacaacattatactactacagagatagatctaaatgatattatgcaaaatatagaacctacatatcctcatgggctaagagttgtttatgaaagtttacccttttataaagcagagaaaatagtaaatcttatatcaggtacaaaatctataactaacatactggaaaaaacttctgccatagacttaacagatattgatagagccactgagatgatgaggaaaaacataactttgcttataaggatacttccattggattgtaacagagataaaagagagatattgagtatggaaaacctaagtattactgaattaagcaaatatgttagggaaagatcttggtctttatccaatatagttggtgttacatcacccagtatcatgtatacaatggacatcaaatatactacaagcactatatctagtggcataattatagagaaatataatgttaacagtttaacacgtggtgagagaggacccactaaaccatgggttggttcatctacacaagagaaaaaaacaatgccagtttataatagacaagtcttaaccaaaaaacagagagatcaaatagatctattagcaaaattggattgggtgtatgcatctatagataacaaggatgaattcatggaagaactcagcataggaacccttgggttaacatatgaaaaggccaagaaattatttccacaatatttaagtgtcaattatttgcatcgccttacagtcagtagtagaccatgtgaattccctgcatcaataccagcttatagaacaacaaattatcactttgacactagccctattaatcgcatattaacagaaaagtatggtgatgaagatattgacatagtattccaaaactgtataagctttggccttagtttaatgtcagtagtagaacaatttactaatgtatgtcctaacagaattattctcatacctaagcttaatgagatacatttgatgaaacctcccatattcacaggtgatgttgatattcacaagttaaaacaagtgatacaaaaacagcatatgtttttaccagacaaaataagtttgactcaatatgtggaattattcttaagtaataaaacactcaaatctggatctcatgttaattctaatttaatattggcacataaaatatctgactattttcataatacttacattttaagtactaatttagctggacattggattctgattatacaacttatgaaagattctaaaggtatttttgaaaaagattggggagagggatatataactgatcatatgtttattaatttgaaagttttcttcaatgcttataagacctatctcttgtgttttcataaaggttatggcaaagcaaagctggagtgtgatatgaacacttcagatcttctatgtgtattggaattaatagacagtagttattggaagtctatgtctaaggtatttttagaacaaaaagttatcaaatacattcttagccaagatgcaagtttacatagagtaaaaggatgtcatagcttcaaattatggtttcttaaacgtcttaatgtagcagaattcacagtttgcccttgggttgttaacatagattatcatccaacacatatgaaagcaatattaacttatatagatcttgttagaatgggattgataaatatagatagaatacacattaaaaataaacacaaattcaatgatgaattttatacttctaatctcttctacattaattataacttctcagataatactcatctattaactaaacatataaggattgctaattctgaattagaaaataattacaacaaattatatcatcctacaccagaaaccctagagaatatactagccaatccgattaaaagtaatgacaaaaagacactgaatgactattgtataggtaaaaatgttgactcaataatgttaccattgttatctaataagaagcttattaaatcgtctgcaatgattagaaccaattacagcaaacaagatttgtataatttattccctatggttgtgattgatagaattatagatcattcaggcaatacagccaaatccaaccaactttacactactacttcccaccaaatatccttagtgcacaatagcacatcactttactgcatgcttccttggcatcatattaatagattcaattttgtatttagttctacaggttgtaaaattagtatagagtatattttaaaagatcttaaaattaaagatcccaattgtatagcattcataggtgaaggagcagggaatttattattgcgtacagtagtggaacttcatcctgacataagatatatttacagaagtctgaaagattgcaatgatcatagtttacctattgagtttttaaggctgtacaatggacatatcaacattgattatggtgaaaatttgaccattcctgctacagatgcaaccaacaacattcattggtcttatttacatataaagtttgctgaacctatcagtctttttgtctgtgatgccgaattgtctgtaacagtcaactggagtaaaattataatagaatggagcaagcatgtaagaaagtgcaagtactgttcctcagttaataaatgtatgttaatagtaaaatatcatgctcaagatgatattgatttcaaattagacaatataactatattaaaaacttatgtatgcttaggcagtaagttaaagggatcggaggtttacttagtccttacaataggtcctgcgaatatattcccagtatttaatgtagtacaaaatgctaaattgatactatcaagaaccaaaaatttcatcatgcctaagaaagctgataaagagtctattgatgcaaatattaaaagtttgataccctttctttgttaccctataacaaaaaaaggaattaatactgcattgtcaaaactaaagagtgttgttagtggagatatactatcatattctatagctggacgtaatgaagttttcagcaataaacttataaatcataagcatatgaacatcttaaaatggttcaatcatgttttaaatttcagatcaacagaactaaactataaccatttatatatggtagaatctacatatccttacctaagtgaattgttaaacagcttgacaaccaatgaacttaaaaaactgattaaaatcacaggtagtctgttatacaactttcataatgaataatgaataaagatcttataataaaaattcccatagctatacactaacactgtattcaattatagttattaaaaattaaaaatcatataattttttaaataacttttagtgaactaatcctaaagttatcattttaatcttggaggaataaatttaaaccctaatctaattggtttatatgtgtattaactaaattacgagatattagtttttgacactttttttctcgt

SEQ ID NO: 2 - DNA, 15111 bp, Human respiratory syncytial virus
acgggaaaaaatgcgtacaacaaacttgcataaaccaaaaaaatggggcaaataagaatttgataagtaccacttaaatttaactcccttggttagagatgggcagcaattcattgagtatgataaaagtcagattgcaaaatctattcgataatgacgaagtggcactattaaaaattacatgttataccgataaattgatacatctaactaatgcattagctaaagctgtaatacatacaattaaacttaatggaatagtgtttgtacatgtaattacatctagtgatatatgccctaataataatatcgtagtcaagtctaattttacaacaatgccagtgttacaaaatggcggatatatttgggaaatgatggaattgacacattgctcacaacctaatggtctattagacgataattgcgaaattaaatttagtaagaaattatccgatagtacaatgactaattatatgaatcaattatccgaattgttaggtttcgatcttaatccataaattataattaatatcaactagcaaatcaatgtcactaacaccattagttaatataaaacttaacagaagacaaaaatggggcaaataaatcaattcagccaacccaaccatggacacaacccacaatgataatacaccacaaagactgatgattaccgatatgagaccgttgtcacttgagacaattataactagcctaactagagatataataacacataaatttatatatctgattaatcacgaatgcatcgtgaggaaattggacgaaagacaggccacatttacattcttagtcaattacgaaatgaaactattgcataaggtaggctcaactaagtataagaaatataccgaatataacactaaatacggaacattcccaatgcctatattcataaatcacgacgggtttctcgaatgcataggcataaaacctacaaaacatacacccataatctataaatacgatcttaacccataaatttcaacacaatattcacacaatctaaaacaacaactctatgcataactatactccatagtccagatggagcctgaaaattatagtaatttaaaacttaaggagagatataagatagaagatggggcaaatacaaccatggctcttagcaaagtcaagttgaatgatacattgaataaagatcaattactatctagctcgaaatatactatccaacggtctacaggcgattcaatagatacacctaattacgatgtgcaaaaacatattaataaattgtgtggtatgttattgattaccgaagacgcaaatcataaatttacagggttaatcggtatgttatacgctatgtctagattaggtagggaagatacaattaaaatacttagagacgcaggatatcacgttaaagctaacggagtagacgtaactacacatagacaggatattaacggtaaggaaatgaaattcgaagtgttaacactcgctagcttaactaccgaaatacaaattaatatcgaaatcgaatcacgtaaatcttataagaaaatgcttaaagaaatgggcgaagtcgcacccgaatatagacacgatagtcccgattgtggtatgattatactatgtatagccgcattagtgataactaagttggccgcaggcgatagatccggattaaccgcagtgatacgtagagcgaataacgtacttaaaaacgaaatgaaacggtataagggtctattaccaaaagatatagcgaatagtttttacgaagtattcgaaaaacatccacattttatagacgtttttgtgcatttcggaatcgcacaatctagtactagaggaggatctagggttgagggtatattcgcaggattgtttatgaacgcatacggagcaggtcaagtcatgcttagatggggagtactcgcaaaatccgttaaaaatattatgttaggacacgctagcgtacaagccgaaatggaacaagtcgttgaggtatacgaatacgcacaaaaattaggtggagaagcaggattttatcatatactgaataatcctaaagctagtctattaagcttaacacaatttccacatttttctagcgtagtgttaggtaacgcagctggcctaggcataatgggcgaatataggggtacacctagaaatcaggatctatatgacgcagctaaagcatacgctgaacaattgaaagagaatggagtgataaattattccgtactcgatctaacagccgaagagttggaggcaattaaacatcaattgaatccgaaagataatgacgttgagttgtgagttaataaaaaatggggcaaataaatcatcatggaaaagtttgctcctgaattccatggagaagacgcaaataatagggcaacaaaattcttagagtcaatcaagggtaagtttacaagtccaaaagatccaaagaagaaagatagtataataagcgtaaactcaattgatatcgaggtgacaaaggaatcacctataacatctaatagtacaataataaatcccactaacgaaacagacgataccgcaggcaataaacctaattatcaacggaaacccttagtgtcattcaaagaagatccaacacctagtgataatccctttagtaaattgtataaggaaacaatcgaaacattcgataataacgaagaagaatcatcatactcatacgaagagataaacgatcagactaacgataatataaccgctagactagatagaatagacgaaaaactatctgaaatactaggtatgttacacacactagtagtcgcatctgccggacctacaagtgctagagatgggataagggatgcaatggtagggttaagggaagaaatgatagagaaaattagaaccgaagcattaatgactaacgatagactcgaagcaatggctagacttagaaacgaagaatccgaaaagatggcaaaagatacatctgacgaagtgtcacttaatcctactagcgaaaaattgaataatctattagagggaaacgatagtgataacgatctatcactcgaagatttctgattagttaccaatcttcacatcaacacacaataccaacagaagaccaacaaactaaccaacccaatcatccaaccaaacatccatccgccaatcagccaaacagccaacaaaacaaccagccaatccaaaactaaccacccggaaaaaatctataatatagttacaaaaaaaggaaagggtggggcaaatatggaaacatacgtgaacaagcttcacgaaggatcaacatatacagctgcagtccaatataacgtactcgaaaaagacgacgatcccgctagcctaacaatatgggtcccaatgtttcaatctagtatgcccgctgatctattaatcaaagaactagctaacgttaacatactagtcaaacaaattagtacacctaagggaccctcacttagagtgatgattaatagtagatccgcagtcctagcacaaatgcctagtaagtttacaatatgtgctaacgtaagcttagacgaacgatcaaaactagcatacgatgtgacaacaccatgcgaaatcaaagcatgttcattgacatgtcttaaatcaaagaatatgctaacaacagtcaaagatctaacaatgaaaacacttaatcccacacacgatataatcgcactatgcgaattcgaaaatatagtgactagtaagaaagtgataatccctacataccttagatcaatatccgttagaaataaggatctgaatacactcgaaaatataacaacaaccgaattcaaaaacgctataactaacgctaagataatcccttactccggactattgttagtgataaccgtaaccgataataagggagcattcaaatacataaaaccccaatcccaatttatagtcgatttaggcgcatacttagaaaaagaatcaatctattacgttacaactaattggaaacataccgctactagattcgcaatcaaacctatggaagattaacctttttcctctacatcagtgtgttaattcatacaaactttctacctacattcttcacttcaccatcacaatcacaaacactctgtggttcaaccaatcaaacaaaacttatctgaagtcccagatcatcccaagtcattgtttatcagatctagtactcaaataagttaataaaaaatatacacatggggcaaataatcattggaggaaatccaactaatcacaatatctgttaacatagacaagtccacacaccatacagaatcaaccaatggaaaatacatccataacaatagaattctctagcaaattttggccttactttacactaatacacatgataactacaatcatatccctattaatcataatctcaattatgatcgcaatccttaacaaactatgtgagtataacgtattccataacaaaacattcgaattgccaagagctcgagtgaatacctgataaagtagttaattaaaaatagtcataacaatgaactaggatatcaagactaacaataacattggggcaaatgcaaacatgtccaaaaacaaggaccaacgcaccgctaagacattagaaaggacctgggacactctcaatcatttattattcatatcatcgtgcttatataagttaaatcttaaatctgtagcacaaatcacattatccattctggcaatgataatctcaacttcacttataattgcagccatcatattcatagcctcggcaaaccacaaagtcacaccaacaactgcaatcatacaagatgcaacaagccagatcaagaacacaaccccaacatacctcacccagaatcctcagcttggaatcagtccctctaatccgtctgaaattacatcacaaatcaccaccatactagcttcaacaacaccaggagtcaagtcaaccctgcaatccacaacagtcaagaccaaaaacacaacaacaactcaaacacaacccagcaagcccaccacaaaacaacgccaaaacaaaccaccaagcaaacccaataatgattttcactttgaagtgttcaactttgtaccctgcagcatatgcagcaacaatccaacctgctgggctatctgcaaaagaataccaaacaaaaaaccaggaaagaaaaccactaccaagcccacaaaaaaaccaaccctcaagacaaccaaaaaagatcccaaacctcaaaccactaaatcaaaggaagtacccaccaccaagcccacagaagagccaaccatcaacaccaccaaaacaaacatcataactacactactcacctccaacaccacaggaaatccagaactcacaagtcaaatggaaaccttccactcaacttcctccgaaggcaatccaagcccttctcaagtctctacaacatccgagtacccatcacaaccttcatctccacccaacacaccacgccagtagttacttaaaaacatattatcacaaaaggccttgaccaacttaaacagaatcaaaataaactctggggcaaataacaatggagttgctaatcctcaaagcaaatgcaattaccacaatcctcactgcagtcacattttgttttgcttctggtcaaaacatcactgaagaattttatcaatcaacatgcagtgcagttagcaaaggctatcttagtgctctgagaactggttggtataccagtgttataactatagaattaagtaatatcaagaaaaataagtgtaatggaacagatgctaaggtaaaattgataaaacaagaattagataaatataaaaatgctgtaacagaattgcagttgctcatgcaaagcacacaagcaacaaacaatcgagccagaagagaactaccaaggtttatgaattatacactcaacaatgccaaaaaaaccaatgtaacattaagcaagaaaaggaaaagaagatttcttggttttttgttaggtgttggatctgcaatcgccagtggcgttgctgtatctaaggtcctgcacctagaaggggaagtgaacaagatcaaaagtgctctactatccacaaacaaggctgtagtcagcttatcaaatggagttagtgttttaaccagcaaagtgttagacctcaaaaactatatagataaacaattgttacctattgtgaacaagcaaagctgcagcatatcaaatatagaaactgtgatagagttccaacaaaagaacaacagactactagagattaccagggaatttagtgttaatgcaggcgtaactacacctgtaagcacttacatgttaactaatagtgaattattgtcattaatcaatgatatgcctataacaaatgatcagaaaaagttaatgtccaacaatgttcaaatagttagacagcaaagttactctatcatgtccataataaaagaggaagtcttagcatatgtagtacaattaccactatatggtgttatagatacaccctgttggaaactacacacatcccctctatgtacaaccaacacaaaagaagggtccaacatctgtttaacaagaactgacagaggatggtactgtgacaatgcaggatcagtatctttcttcccacaagctgaaacatgtaaagttcaatcaaatcgagtattttgtgacacaatgaacagtttaacattaccaagtgaagtaaatctctgcaatgttgacatattcaaccccaaatatgattgtaaaattatgacttcaaaaacagatgtaagcagctccgttatcacatctctaggagccattgtgtcatgctatggcaaaactaaatgtacagcatccaataaaaatcgtggaatcataaagacattttctaacgggtgcgattatgtatcaaataaaggggtggacactgtgtctgtaggtaacacattatattatgtaaataagcaagaaggtaaaagtctctatgtaaaaggtgaaccaataataaatttctatgacccattagtattcccctctgatgaatttgatgcatcaatatctcaagtcaacgagaagattaaccagagcctagcatttattcgtaaatccgatgaattattacataatgtaaatgctggtaaatccaccacaaatatcatgataactactataattatagtgattatagtaatattgttatcattaattgctgttggactgctcttatactgtaaggccagaagcacaccagtcacactaagcaaagatcaactgagtggtataaataatattgcatttagtaactaaataaaaatagcacctaatcatgttcttacaatggtttactatctgctcatagacaacccatctgtcattggattttcttaaaatctgaacttcatcgaaactctcatctataaaccatctcacttacactatttaagtagattcctagtttatagttatataaaacacaattgcatgccagattaacttaccatctgtaaaaatgaaaactggggcaaatatgtcacgaaggaatccttgcaaatttgaaattcgaggtcattgcttaaatggtaagaggtgtcattttagtcataattattttgaatggccaccccatgcactgcttgtaagacaaaactttatgttaaacagaatacttaagtctatggataaaagtatagataccttatcagaaataagtggagctgcagagttggacagaacagaagagtatgctcttggtgtagttggagtgctagagagttatataggatcaataaacaatataactaaacaatcagcatgtgttgccatgagcaaactcctcactgaactcaatagtgatgatatcaaaaagctgagggacaatgaagagctaaattcacccaagataagagtgtacaatactgtcatatcatatattgaaagcaacaggaaaaacaataaacaaactatccatctgttaaaaagattgccagcagacgtattgaagaaaaccatcaaaaacacattggatatccataagagcataaccatcaacaacccaaaagaatcaactgttagtgatacaaatgaccatgccaaaaataatgatactacctgacaaatatccttgtagtataacttccatactaataacaagtagatgtagagttactatgtataatcaaaagaacacactatatttcaatcaaaacaacccaaataaccatatgtactcaccgaatcaaacattcaatgaaatccattggacctctcaagaattgattgacacaattcaaaattttctacaacatctaggtattattgaggatatatatacaatatatatattagtgtcataacactcaattctaacactcaccacatcgttacattattaattcaaacaattcaagttgtgggacaaaatggatcccattattaatggaaattctgctaatgtttatctaaccgatagttatttaaaaggtgttatctctttctcagagtgtaatgctttaggaagttacatattcaatggtccttatctcaaaaatgattataccaacttaattagtagacaaaatccattaatagaacacatgaatctaaagaaactaaatataacacagtccttaatatctaagtatcataaaggtgaaataaaattagaagaacctacttattttcagtcattacttatgacatacaagagtatgacctcgtcagaacagattgctaccactaatttacttaaaaagataataagaagagctatagaaataagtgatgtcaaagtctatgctatattgaataaactagggcttaaagaaaaggacaagattaaatccaacaatggacaagatgaagacaactcagttattacgaccataatcaaagatgatatactttcagctgttaaagataatcaatctcatcttaaagcagacaaaaatcactctacaaaacaaaaagacacaatcaaaacaacactcttgaagaaattgatgtgttcaatgcaacatcctccatcatggttaatacattggtttaacttatacacaaaattaaacaacatattaacacagtatcgatcaaatgaggtaaaaaaccatgggtttacattgatagataatcaaactcttagtggatttcaatttattttgaaccaatatggttgtatagtttatcataaggaactcaaaagaattactgtgacaacctataatcaattcttgacatggaaagatattagccttagtagattaaatgtttgtttaattacatggattagtaactgcttgaacacattaaataaaagcttaggcttaagatgcggattcaataatgttatcttgacacaactattcctttatggagattgtatactaaagctatttcacaatgaggggttctacataataaaagaggtagagggatttattatgtctctaattttaaatataacagaagaagatcaattcagaaaacgattttataatagtatgctcaacaacatcacagatgctgctaataaagctcagaaaaatctgctatcaagagtatgtcatacattattagataagacagtgtccgataatataataaatggcagatggataattctattaagtaagttccttaaattaattaagcttgcaggtgacaataaccttaacaatctgagtgaactatattttttgttcagaatatttggacacccaatggtagatgaaagacaagccatggatgctgttaaaattaattgcaatgagaccaaattttacttgttaagcagtctgagtatgttaagaggtgcctttatatatagaattataaaagggtttgtaaataattacaacagatggcctactttaagaaatgctattgttttacccttaagatggttaacttactataaactaaacacttatccttctttgttggaacttacagaaagagatttgattgtgttatcaggactacgtttctatcgtgagtttcggttgcctaaaaaagtggatcttgaaatgattataaatgataaagctatatcacctcctaaaaatttgatatggactagtttccctagaaattacatgccatcacacatacaaaactatatagaacatgaaaaattaaaattttccgagagtgataaatcaagaagagtattagagtattatttaagagataacaaattcaatgaatgtgatttatacaactgtgtagttaatcaaagttatctcaacaaccctaatcatgtggtatcattgacaggcaaagaaagagaactcagtgtaggtagaatgtttgcaatgcaaccgggaatgttcagacaggttcaaatattggcagagaaaatgatagctgaaaacattttacaattctttcctgaaagtcttacaagatatggtgatctagaactacaaaaaatattagaactgaaagcaggaataagtaacaaatcaaatcgctacaatgataattacaacaattacattagtaagtgctctatcatcacagatctcagcaaattcaatcaagcatttcgatatgaaacgtcatgtatttgtagtgatgtgctggatgaactgcatggtgtacaatctctattttcctggttacatttaactattcctcatgtcacaataatatgcacatataggcatgcacccccctatataggagatcatattgtagatcttaacaatgtagatgaacaaagtggattatatagatatcacatgggtggcatcgaagggtggtgtcaaaaactatggaccatagaagctatatcactattggatctaatatctctcaaagggaaattctcaattactgctttaattaatggtgacaatcaatcaatagatataagcaaaccaatcagactcatggaaggtcaaactcatgctcaagcagattatttgctagcattaaatagccttaaattactgtataaagagtatgcaggcataggccacaaattaaaaggaactgagacttatatatcacgagatatgcaatttatgagtaaaacaattcaacataacggtgtatattacccagctagtataaagaaagtcctaagagtgggaccgtggataaacactatacttgatgatttcaaagtgagtctagaatctataggtagtttgacacaagaattagaatatagaggtgaaagtctattatgcagtttaatatttagaaatgtatggttatataatcagattgctctacaattaaaaaatcatgcattatgtaacaataaactatatttggacatattaaaggttctgaaacacttaaaaaccttttttaatcttgataatattgatacagcattaacattgtatatgaatttacccatgttatttggtggtggtgatcccaacttgttatatcgaagtttctatagaagaactcctgacttcctcacagaggctatagttcactctgtgttcatacttagttattatacaaaccatgacttaaaagataaacttcaagatctgtcagatgatagattgaataagttcttaacatgcataatcacgtttgacaaaaaccctaatgctgaattcgtaacattgatgagagatcctcaagctttagggtctgagagacaagctaaaattactagcgaaatcaatagactggcagttacagaggttttgagtacagctccaaacaaaatattctccaaaagtgcacaacattatactactacagagatagatctaaatgatattatgcaaaatatagaacctacatatcctcatgggctaagagttgtttatgaaagtttacccttttataaagcagagaaaatagtaaatcttatatcaggtacaaaatctataactaacatactggaaaaaacttctgccatagacttaacagatattgatagagccactgagatgatgaggaaaaacataactttgcttataaggatacttccattggattgtaacagagataaaagagagatattgagtatggaaaacctaagtattactgaattaagcaaatatgttagggaaagatcttggtctttatccaatatagttggtgttacatcacccagtatcatgtatacaatggacatcaaatatactacaagcactatatctagtggcataattatagagaaatataatgttaacagtttaacacgtggtgagagaggacccactaaaccatgggttggttcatctacacaagagaaaaaaacaatgccagtttataatagacaagtcttaaccaaaaaacagagagatcaaatagatctattagcaaaattggattgggtgtatgcatctatagataacaaggatgaattcatggaagaactcagcataggaacccttgggttaacatatgaaaaggccaagaaattatttccacaatatttaagtgtcaattatttgcatcgccttacagtcagtagtagaccatgtgaattccctgcatcaataccagcttatagaacaacaaattatcactttgacactagccctattaatcgcatattaacagaaaagtatggtgatgaagatattgacatagtattccaaaactgtataagctttggccttagtttaatgtcagtagtagaacaatttactaatgtatgtcctaacagaattattctcatacctaagcttaatgagatacatttgatgaaacctcccatattcacaggtgatgttgatattcacaagttaaaacaagtgatacaaaaacagcatatgtttttaccagacaaaataagtttgactcaatatgtggaattattcttaagtaataaaacactcaaatctggatctcatgttaattctaatttaatattggcacataaaatatctgactattttcataatacttacattttaagtactaatttagctggacattggattctgattatacaacttatgaaagattctaaaggtatttttgaaaaagattggggagagggatatataactgatcatatgtttattaatttgaaagttttcttcaatgcttataagacctatctcttgtgttttcataaaggttatggcaaagcaaagctggagtgtgatatgaacacttcagatcttctatgtgtattggaattaatagacagtagttattggaagtctatgtctaaggtatttttagaacaaaaagttatcaaatacattcttagccaagatgcaagtttacatagagtaaaaggatgtcatagcttcaaattatggtttcttaaacgtcttaatgtagcagaattcacagtttgcccttgggttgttaacatagattatcatccaacacatatgaaagcaatattaacttatatagatcttgttagaatgggattgataaatatagatagaatacacattaaaaataaacacaaattcaatgatgaattttatacttctaatctcttctacattaattataacttctcagataatactcatctattaactaaacatataaggattgctaattctgaattagaaaataattacaacaaattatatcatcctacaccagaaaccctagagaatatactagccaatccgattaaaagtaatgacaaaaagacactgaatgactattgtataggtaaaaatgttgactcaataatgttaccattgttatctaataagaagcttattaaatcgtctgcaatgattagaaccaattacagcaaacaagatttgtataatttattccctatggttgtgattgatagaattatagatcattcaggcaatacagccaaatccaaccaactttacactactacttcccaccaaatatccttagtgcacaatagcacatcactttactgcatgcttccttggcatcatattaatagattcaattttgtatttagttctacaggttgtaaaattagtatagagtatattttaaaagatcttaaaattaaagatcccaattgtatagcattcataggtgaaggagcagggaatttattattgcgtacagtagtggaacttcatcctgacataagatatatttacagaagtctgaaagattgcaatgatcatagtttacctattgagtttttaaggctgtacaatggacatatcaacattgattatggtgaaaatttgaccattcctgctacagatgcaaccaacaacattcattggtcttatttacatataaagtttgctgaacctatcagtctttttgtctgtgatgccgaattgtctgtaacagtcaactggagtaaaattataatagaatggagcaagcatgtaagaaagtgcaagtactgttcctcagttaataaatgtatgttaatagtaaaatatcatgctcaagatgatattgatttcaaattagacaatataactatattaaaaacttatgtatgcttaggcagtaagttaaagggatcggaggtttacttagtccttacaataggtcctgcgaatatattcccagtatttaatgtagtacaaaatgctaaattgatactatcaagaaccaaaaatttcatcatgcctaagaaagctgataaagagtctattgatgcaaatattaaaagtttgataccctttctttgttaccctataacaaaaaaaggaattaatactgcattgtcaaaactaaagagtgttgttagtggagatatactatcatattctatagctggacgtaatgaagttttcagcaataaacttataaatcataagcatatgaacatcttaaaatggttcaatcatgttttaaatttcagatcaacagaactaaactataaccatttatatatggtagaatctacatatccttacctaagtgaattgttaaacagcttgacaaccaatgaacttaaaaaactgattaaaatcacaggtagtctgttatacaactttcataatgaataatgaataaagatcttataataaaaattcccatagctatacactaacactgtattcaattatagttattaaaaattaaaaatcatataattttttaaataacttttagtgaactaatcctaaagttatcattttaatcttggaggaataaatttaaaccctaatctaattggtttatatgtgtattaactaaattacgagatattagtttttgacactttttttctcgt

SEQ ID NO: 3 - DNA, 15111 bp, Human respiratory syncytial virus
acgggaaaaaatgcgtacaacaaacttgcataaaccaaaaaaatggggcaaataagaatttgataagtaccacttaaatttaactcccttggttagagatgggcagcaattcattgagtatgataaaagttagattacaaaatttgtttgacaatgatgaagtagcattgttaaaaataacatgctatactgataaattaatacatttaactaatgctttggctaaggcagtgatacatacaatcaaattgaatggcattgtgtttgtgcatgttattacaagtagtgatatttgccctaataataatattgtagtaaaatccaatttcacaacaatgccagtactacaaaatggaggttatatatgggaaatgatggaattaacacattgctctcaacctaatggtctactagatgacaattgtgaaattaaattctccaaaaaactaagtgattcaacaatgaccaattatatgaatcaattatctgaattacttggatttgatcttaatccataaattataattaatatcaactagcaaatcaatgtcactaacaccattagttaatataaaacttaacagaagacaaaaatggggcaaataaatcaattcagccaacccaaccatggacacaacccacaatgataatacaccacaaagactgatgatcacagacatgagaccgttgtcacttgagaccataataacatcactaaccagagacatcataacacacaaatttatatacttgataaatcatgaatgcatagtgagaaaacttgatgaaagacaggccacatttacattcctggtcaactatgaaatgaaactattacacaaagtaggaagcactaaatataaaaaatatactgaatacaacacaaaatatggcactttccctatgccaatattcatcaatcatgatgggttcttagaatgcattggcattaagcctacaaagcatactcccataatatacaagtatgatctcaatccataaatttcaacacaatattcacacaatctaaaacaacaactctatgcataactatactccatagtccagatggagcctgaaaattatagtaatttaaaacttaaggagagatataagatagaagatggggcaaatacaaccatggctcttagcaaagtcaagttgaatgatacactcaacaaagatcaacttctgtcatccagcaaatacaccatccaacggagcacaggagatagtattgatactcctaattatgatgtgcagaaacacatcaataagttatgtggcatgttattaatcacagaagatgctaatcataaattcactgggttaataggtatgttatatgcgatgtctaggttaggaagagaagacaccataaaaatactcagagatgcgggatatcatgtaaaagcaaatggagtagatgtaacaacacatcgtcaagacattaatggaaaagaaatgaaatttgaagtgttaacattggcaagcttaacaactgaaattcaaatcaacattgagatagaatctagaaaatcctacaaaaaaatgctaaaagaaatgggagaggtagctccagaatacaggcatgactctcctgattgtgggatgataatattatgtatagcagcattagtaataactaaattagcagcaggggacagatctggtcttacagccgtgattaggagagctaataatgtcctaaaaaatgaaatgaaacgttacaaaggcttactacccaaggacatagccaacagcttctatgaagtgtttgaaaaacatccccactttatagatgtttttgttcattttggtatagcacaatcttctaccagaggtggcagtagagttgaagggatttttgcaggattgtttatgaatgcctatggtgcagggcaagtgatgttacggtggggagtcttagcaaaatcggttaaaaatattatgttaggacatgctagtgtgcaagcagaaatggaacaagttgttgaggtttatgaatatgcccaaaaattgggtggtgaagcaggattctaccatatattgaacaacccaaaagcatcattattatctttgactcaatttcctcacttctccagtgtagtattaggcaatgctgctggcctaggcataatgggagagtacagaggtacaccgaggaatcaagatctatatgatgcagcaaaggcatatgctgaacaactcaaagaaaatggtgtgattaactacagtgtactagacttgacagcagaagaactagaggctatcaaacatcagcttaatccaaaagataatgatgtagagctttgagttaataaaaaatggggcaaataaatcatcatggaaaagtttgctcctgaattccatggagaagatgcaaacaacagggctactaaattcctagaatcaataaagggcaaattcacatcacccaaagatcccaagaaaaaagatagtatcatatctgtcaactcaatagatatagaagtaaccaaagaaagccctataacatcaaattcaactattatcaacccaacaaatgagacagatgatactgcagggaacaagcccaattatcaaagaaaacctctagtaagtttcaaagaagaccctacaccaagtgataatcccttttctaaactatacaaagaaaccatagaaacatttgataacaatgaagaagaatccagctattcatacgaagaaataaatgatcagacaaacgataatataacagcaagattagataggattgatgaaaaattaagtgaaatactaggaatgcttcacacattagtagtggcaagtgcaggacctacatctgctcgggatggtataagagatgccatggttggtttaagagaagaaatgatagaaaaaatcagaactgaagcattaatgaccaatgacagattagaagctatggcaagactcaggaatgaggaaagtgaaaagatggcaaaagacacatcagatgaagtgtctctcaatccaacatcagagaaattgaacaacctattggaagggaatgatagtgacaatgatctatcacttgaagatttctgattagttaccaatcttcacatcaacacacaataccaacagaagaccaacaaactaaccaacccaatcatccaaccaaacatccatccgccaatcagccaaacagccaacaaaacaaccagccaatccaaaactaaccacccggaaaaaatctataatatagttacaaaaaaaggaaagggtggggcaaatatggaaacatacgtgaacaagcttcacgaaggctccacatacacagctgctgttcaatacaatgtcttagaaaaagacgatgaccctgcatcacttacaatatgggtgcccatgttccaatcatctatgccagcagatttacttataaaagaactagctaatgtcaacatactagtgaaacaaatatccacacccaagggaccttcactaagagtcatgataaactcaagaagtgcagtgctagcacaaatgcccagcaaatttaccatatgcgctaatgtgtccttggatgaaagaagcaaactagcatatgatgtaaccacaccctgtgaaatcaaggcatgtagtctaacatgcctaaaatcaaaaaatatgttgactacagttaaagatctcactatgaagacactcaaccctacacatgatattattgctttatgtgaatttgaaaacatagtaacatcaaaaaaagtcataataccaacatacctaagatccatcagtgtcagaaataaagatctgaacacacttgaaaatataacaaccactgaattcaaaaatgctatcacaaatgcaaaaatcatcccttactcaggattactattagtcatcacagtgactgacaacaaaggagcattcaaatacataaagccacaaagtcaattcatagtagatcttggagcttacctagaaaaagaaagtatatattatgttaccacaaattggaagcacacagctacacgatttgcaatcaaacccatggaagattaacctttttcctctacatcagtgtgttaattcatacaaactttctacctacattcttcacttcaccatcacaatcacaaacactctgtggttcaaccaatcaaacaaaacttatctgaagtcccagatcatcccaagtcattgtttatcagatctagtactcaaataagttaataaaaaatatacacatggggcaaataatcattggaggaaatccaactaatcacaatatctgttaacatagacaagtccacacaccatacagaatcaaccaatggaaaatacatccataacaatagaattctcaagcaaattctggccttactttacactaatacacatgatcacaacaataatctctttgctaatcataatctccatcatgattgcaatactaaacaaactttgtgaatataacgtattccataacaaaacctttgagttaccaagagctcgagttaatacttgataaagtagttaattaaaaatagtcataacaatgaactaggatatcaagactaacaataacattggggcaaatgcaaacatgtccaaaaacaaggaccaacgcaccgctaaaacactcgaaaggacatgggatacccttaatcacctattattcataagctcatgcttatataaattgaaccttaaatccgtcgcacagataaccctatcaatactcgcaatgataatctcaacaagcttaatcatagccgcaataatctttatcgctagcgctaaccataaggtaaccccaacaaccgcaattatacaggacgcaacatcccaaatcaaaaacacaaccccaacatacttaacccaaaacccacaactcggaatctcaccctctaacccatccgaaattacctcacagattacaacgatactcgcaagtacaacccccggagtcaaatcgacactccaatcgacaaccgtaaagactaagaatacaacaacaacccaaacccaacctagtaagcctacaactaagcaacgccaaaacaaacctccctctaaaccgaataacgattttcacttcgaagtgttcaatttcgtaccatgctcaatttgctctaataacccaacatgctgggccatatgcaaacgcatcccaaacaagaaacccggaaagaaaacaaccactaagccaacaaagaaaccaacccttaagacaaccaagaaagatccaaaaccccaaacaactaagtctaaagaggtcccaacaactaagccaaccgaagagccaacaatcaatacaactaagactaatataatcacaaccttactgacatctaacacaaccggaaatcccgaactgacatcccaaatggaaacctttcactcaacctctagcgaaggcaatccctcaccatcccaagtctcaaccactagcgaatacccatcccaacctagctcacctcccaatacccctagacagtagttacttaaaaacatattatcacaaaaggccttgaccaacttaaacagaatcaaaataaactctggggcaaataacaatggagttgctaatcctcaaagcaaatgcaatcacaacaatactaacagccgttacattttgtttcgctagcggacaaaacataaccgaagagttttatcaatctacatgttccgccgtaagtaaggggtatctatccgcacttagaaccggatggtatactagcgtaataacaatcgaactatctaatataaagaagaataagtgtaacggtacagacgctaaggttaaattgattaaacaggaactcgataagtataaaaacgccgtaaccgaattgcaattgttaatgcaatctacacaagctactaataatagggctagacgtgaattgcctagatttatgaattatacacttaataacgctaagaaaactaacgttacactatctaagaaacgaaaacgtagattcttagggtttttactcggagtcggttccgcaatcgctagcggagtcgccgtaagtaaagtgttacacctcgaaggcgaagtgaataagataaaatccgcactattatcaactaataaggcagtcgttagcctatctaacggagtcagcgtattgacatctaaagtgttagacttaaagaattatatagataagcaattgttaccaatcgttaataaacaatcatgttcaatatccaatatcgaaaccgtaatcgaatttcaacagaagaataatagattactcgaaattactagagaatttagcgtaaacgctggcgtaacaacacccgtaagtacatatatgttaactaattccgaactgttaagcttaattaacgatatgccaattactaacgatcagaagaaattgatgtctaataacgtacaaatcgttagacagcaatcatattcaattatgtcaattataaaagaagaggtactcgcatacgtagtgcaattacccctatatggcgtaatagatacaccatgttggaaattgcatacaagtccactatgtacaactaatacaaaagagggatctaatatatgcttaactagaaccgatagggggtggtattgcgataacgcaggtagcgtaagtttctttccacaagccgaaacatgtaaagtgcaatctaatagagtgttttgcgatacaatgaatagcttaacactacctagcgaagtcaatctatgtaacgtcgatatattcaatcctaaatatgattgcaaaattatgactagtaagactgacgtaagtagtagcgtaattactagtctcggtgcaatagtgtcatgttatggtaagactaagtgtaccgctagcaataagaatagggggataataaaaacatttagtaacggttgcgattacgttagtaataagggagtcgataccgtaagcgtaggtaatacactatattatgttaataaacaggaaggtaagtcattatacgttaaaggcgaacctataattaatttttacgatccattagtgtttccatccgacgaattcgacgctagtataagtcaggtaaacgaaaagattaaccaatcactcgcattcatacgaaaatccgacgaactgttacacaacgttaacgcaggtaagagtacaactaacataatgataacaacaattataatcgttataatcgttatactgttaagcttaatcgcagtcggattactgttatattgtaaagctagatcaacacccgtaacactatctaaagaccaattatccggtataaataatatcgcattctcaaactaaataaaaatagcacctaatcatgttcttacaatggtttactatctgctcatagacaacccatctgtcattggattttcttaaaatctgaacttcatcgaaactctcatctataaaccatctcacttacactatttaagtagattcctagtttatagttatataaaacacaattgcatgccagattaacttaccatctgtaaaaatgaaaactggggcaaatatgtcacgaaggaatccttgcaaatttgaaattcgaggtcattgcttaaatggtaagaggtgtcattttagtcataattattttgaatggccaccccatgcactgcttgtaagacaaaactttatgttaaacagaatacttaagtctatggataaaagtatagataccttatcagaaataagtggagctgcagagttggacagaacagaagagtatgctcttggtgtagttggagtgctagagagttatataggatcaataaacaatataactaaacaatcagcatgtgttgccatgagcaaactcctcactgaactcaatagtgatgatatcaaaaagctgagggacaatgaagagctaaattcacccaagataagagtgtacaatactgtcatatcatatattgaaagcaacaggaaaaacaataaacaaactatccatctgttaaaaagattgccagcagacgtattgaagaaaaccatcaaaaacacattggatatccataagagcataaccatcaacaacccaaaagaatcaactgttagtgatacaaatgaccatgccaaaaataatgatactacctgacaaatatccttgtagtataacttccatactaataacaagtagatgtagagttactatgtataatcaaaagaacacactatatttcaatcaaaacaacccaaataaccatatgtactcaccgaatcaaacattcaatgaaatccattggacctctcaagaattgattgacacaattcaaaattttctacaacatctaggtattattgaggatatatatacaatatatatattagtgtcataacactcaattctaacactcaccacatcgttacattattaattcaaacaattcaagttgtgggacaaaatggatcccattattaatggaaattctgctaatgtttatctaaccgatagttatttaaaaggtgttatctctttctcagagtgtaatgctttaggaagttacatattcaatggtccttatctcaaaaatgattataccaacttaattagtagacaaaatccattaatagaacacatgaatctaaagaaactaaatataacacagtccttaatatctaagtatcataaaggtgaaataaaattagaagaacctacttattttcagtcattacttatgacatacaagagtatgacctcgtcagaacagattgctaccactaatttacttaaaaagataataagaagagctatagaaataagtgatgtcaaagtctatgctatattgaataaactagggcttaaagaaaaggacaagattaaatccaacaatggacaagatgaagacaactcagttattacgaccataatcaaagatgatatactttcagctgttaaagataatcaatctcatcttaaagcagacaaaaatcactctacaaaacaaaaagacacaatcaaaacaacactcttgaagaaattgatgtgttcaatgcaacatcctccatcatggttaatacattggtttaacttatacacaaaattaaacaacatattaacacagtatcgatcaaatgaggtaaaaaaccatgggtttacattgatagataatcaaactcttagtggatttcaatttattttgaaccaatatggttgtatagtttatcataaggaactcaaaagaattactgtgacaacctataatcaattcttgacatggaaagatattagccttagtagattaaatgtttgtttaattacatggattagtaactgcttgaacacattaaataaaagcttaggcttaagatgcggattcaataatgttatcttgacacaactattcctttatggagattgtatactaaagctatttcacaatgaggggttctacataataaaagaggtagagggatttattatgtctctaattttaaatataacagaagaagatcaattcagaaaacgattttataatagtatgctcaacaacatcacagatgctgctaataaagctcagaaaaatctgctatcaagagtatgtcatacattattagataagacagtgtccgataatataataaatggcagatggataattctattaagtaagttccttaaattaattaagcttgcaggtgacaataaccttaacaatctgagtgaactatattttttgttcagaatatttggacacccaatggtagatgaaagacaagccatggatgctgttaaaattaattgcaatgagaccaaattttacttgttaagcagtctgagtatgttaagaggtgcctttatatatagaattataaaagggtttgtaaataattacaacagatggcctactttaagaaatgctattgttttacccttaagatggttaacttactataaactaaacacttatccttctttgttggaacttacagaaagagatttgattgtgttatcaggactacgtttctatcgtgagtttcggttgcctaaaaaagtggatcttgaaatgattataaatgataaagctatatcacctcctaaaaatttgatatggactagtttccctagaaattacatgccatcacacatacaaaactatatagaacatgaaaaattaaaattttccgagagtgataaatcaagaagagtattagagtattatttaagagataacaaattcaatgaatgtgatttatacaactgtgtagttaatcaaagttatctcaacaaccctaatcatgtggtatcattgacaggcaaagaaagagaactcagtgtaggtagaatgtttgcaatgcaaccgggaatgttcagacaggttcaaatattggcagagaaaatgatagctgaaaacattttacaattctttcctgaaagtcttacaagatatggtgatctagaactacaaaaaatattagaactgaaagcaggaataagtaacaaatcaaatcgctacaatgataattacaacaattacattagtaagtgctctatcatcacagatctcagcaaattcaatcaagcatttcgatatgaaacgtcatgtatttgtagtgatgtgctggatgaactgcatggtgtacaatctctattttcctggttacatttaactattcctcatgtcacaataatatgcacatataggcatgcacccccctatataggagatcatattgtagatcttaacaatgtagatgaacaaagtggattatatagatatcacatgggtggcatcgaagggtggtgtcaaaaactatggaccatagaagctatatcactattggatctaatatctctcaaagggaaattctcaattactgctttaattaatggtgacaatcaatcaatagatataagcaaaccaatcagactcatggaaggtcaaactcatgctcaagcagattatttgctagcattaaatagccttaaattactgtataaagagtatgcaggcataggccacaaattaaaaggaactgagacttatatatcacgagatatgcaatttatgagtaaaacaattcaacataacggtgtatattacccagctagtataaagaaagtcctaagagtgggaccgtggataaacactatacttgatgatttcaaagtgagtctagaatctataggtagtttgacacaagaattagaatatagaggtgaaagtctattatgcagtttaatatttagaaatgtatggttatataatcagattgctctacaattaaaaaatcatgcattatgtaacaataaactatatttggacatattaaaggttctgaaacacttaaaaaccttttttaatcttgataatattgatacagcattaacattgtatatgaatttacccatgttatttggtggtggtgatcccaacttgttatatcgaagtttctatagaagaactcctgacttcctcacagaggctatagttcactctgtgttcatacttagttattatacaaaccatgacttaaaagataaacttcaagatctgtcagatgatagattgaataagttcttaacatgcataatcacgtttgacaaaaaccctaatgctgaattcgtaacattgatgagagatcctcaagctttagggtctgagagacaagctaaaattactagcgaaatcaatagactggcagttacagaggttttgagtacagctccaaacaaaatattctccaaaagtgcacaacattatactactacagagatagatctaaatgatattatgcaaaatatagaacctacatatcctcatgggctaagagttgtttatgaaagtttacccttttataaagcagagaaaatagtaaatcttatatcaggtacaaaatctataactaacatactggaaaaaacttctgccatagacttaacagatattgatagagccactgagatgatgaggaaaaacataactttgcttataaggatacttccattggattgtaacagagataaaagagagatattgagtatggaaaacctaagtattactgaattaagcaaatatgttagggaaagatcttggtctttatccaatatagttggtgttacatcacccagtatcatgtatacaatggacatcaaatatactacaagcactatatctagtggcataattatagagaaatataatgttaacagtttaacacgtggtgagagaggacccactaaaccatgggttggttcatctacacaagagaaaaaaacaatgccagtttataatagacaagtcttaaccaaaaaacagagagatcaaatagatctattagcaaaattggattgggtgtatgcatctatagataacaaggatgaattcatggaagaactcagcataggaacccttgggttaacatatgaaaaggccaagaaattatttccacaatatttaagtgtcaattatttgcatcgccttacagtcagtagtagaccatgtgaattccctgcatcaataccagcttatagaacaacaaattatcactttgacactagccctattaatcgcatattaacagaaaagtatggtgatgaagatattgacatagtattccaaaactgtataagctttggccttagtttaatgtcagtagtagaacaatttactaatgtatgtcctaacagaattattctcatacctaagcttaatgagatacatttgatgaaacctcccatattcacaggtgatgttgatattcacaagttaaaacaagtgatacaaaaacagcatatgtttttaccagacaaaataagtttgactcaatatgtggaattattcttaagtaataaaacactcaaatctggatctcatgttaattctaatttaatattggcacataaaatatctgactattttcataatacttacattttaagtactaatttagctggacattggattctgattatacaacttatgaaagattctaaaggtatttttgaaaaagattggggagagggatatataactgatcatatgtttattaatttgaaagttttcttcaatgcttataagacctatctcttgtgttttcataaaggttatggcaaagcaaagctggagtgtgatatgaacacttcagatcttctatgtgtattggaattaatagacagtagttattggaagtctatgtctaaggtatttttagaacaaaaagttatcaaatacattcttagccaagatgcaagtttacatagagtaaaaggatgtcatagcttcaaattatggtttcttaaacgtcttaatgtagcagaattcacagtttgcccttgggttgttaacatagattatcatccaacacatatgaaagcaatattaacttatatagatcttgttagaatgggattgataaatatagatagaatacacattaaaaataaacacaaattcaatgatgaattttatacttctaatctcttctacattaattataacttctcagataatactcatctattaactaaacatataaggattgctaattctgaattagaaaataattacaacaaattatatcatcctacaccagaaaccctagagaatatactagccaatccgattaaaagtaatgacaaaaagacactgaatgactattgtataggtaaaaatgttgactcaataatgttaccattgttatctaataagaagcttattaaatcgtctgcaatgattagaaccaattacagcaaacaagatttgtataatttattccctatggttgtgattgatagaattatagatcattcaggcaatacagccaaatccaaccaactttacactactacttcccaccaaatatccttagtgcacaatagcacatcactttactgcatgcttccttggcatcatattaatagattcaattttgtatttagttctacaggttgtaaaattagtatagagtatattttaaaagatcttaaaattaaagatcccaattgtatagcattcataggtgaaggagcagggaatttattattgcgtacagtagtggaacttcatcctgacataagatatatttacagaagtctgaaagattgcaatgatcatagtttacctattgagtttttaaggctgtacaatggacatatcaacattgattatggtgaaaatttgaccattcctgctacagatgcaaccaacaacattcattggtcttatttacatataaagtttgctgaacctatcagtctttttgtctgtgatgccgaattgtctgtaacagtcaactggagtaaaattataatagaatggagcaagcatgtaagaaagtgcaagtactgttcctcagttaataaatgtatgttaatagtaaaatatcatgctcaagatgatattgatttcaaattagacaatataactatattaaaaacttatgtatgcttaggcagtaagttaaagggatcggaggtttacttagtccttacaataggtcctgcgaatatattcccagtatttaatgtagtacaaaatgctaaattgatactatcaagaaccaaaaatttcatcatgcctaagaaagctgataaagagtctattgatgcaaatattaaaagtttgataccctttctttgttaccctataacaaaaaaaggaattaatactgcattgtcaaaactaaagagtgttgttagtggagatatactatcatattctatagctggacgtaatgaagttttcagcaataaacttataaatcataagcatatgaacatcttaaaatggttcaatcatgttttaaatttcagatcaacagaactaaactataaccatttatatatggtagaatctacatatccttacctaagtgaattgttaaacagcttgacaaccaatgaacttaaaaaactgattaaaatcacaggtagtctgttatacaactttcataatgaataatgaataaagatcttataataaaaattcccatagctatacactaacactgtattcaattatagttattaaaaattaaaaatcatataattttttaaataacttttagtgaactaatcctaaagttatcattttaatcttggaggaataaatttaaaccctaatctaattggtttatatgtgtattaactaaattacgagatattagtttttgacactttttttctcgt

SEQ ID NO: 4 - DNA, 15111 bp, Human respiratory syncytial virus
acgggaaaaaatgcgtacaacaaacttgcataaaccaaaaaaatggggcaaataagaatttgataagtaccacttaaatttaactcccttggttagagatgggcagcaattcattgagtatgataaaagttagattacaaaatttgtttgacaatgatgaagtagcattgttaaaaataacatgctatactgataaattaatacatttaactaatgctttggctaaggcagtgatacatacaatcaaattgaatggcattgtgtttgtgcatgttattacaagtagtgatatttgccctaataataatattgtagtaaaatccaatttcacaacaatgccagtactacaaaatggaggttatatatgggaaatgatggaattaacacattgctctcaacctaatggtctactagatgacaattgtgaaattaaattctccaaaaaactaagtgattcaacaatgaccaattatatgaatcaattatctgaattacttggatttgatcttaatccataaattataattaatatcaactagcaaatcaatgtcactaacaccattagttaatataaaacttaacagaagacaaaaatggggcaaataaatcaattcagccaacccaaccatggacacaacccacaatgataatacaccacaaagactgatgatcacagacatgagaccgttgtcacttgagaccataataacatcactaaccagagacatcataacacacaaatttatatacttgataaatcatgaatgcatagtgagaaaacttgatgaaagacaggccacatttacattcctggtcaactatgaaatgaaactattacacaaagtaggaagcactaaatataaaaaatatactgaatacaacacaaaatatggcactttccctatgccaatattcatcaatcatgatgggttcttagaatgcattggcattaagcctacaaagcatactcccataatatacaagtatgatctcaatccataaatttcaacacaatattcacacaatctaaaacaacaactctatgcataactatactccatagtccagatggagcctgaaaattatagtaatttaaaacttaaggagagatataagatagaagatggggcaaatacaaccatggctcttagcaaagtcaagttgaatgatacactcaacaaagatcaacttctgtcatccagcaaatacaccatccaacggagcacaggagatagtattgatactcctaattatgatgtgcagaaacacatcaataagttatgtggcatgttattaatcacagaagatgctaatcataaattcactgggttaataggtatgttatatgcgatgtctaggttaggaagagaagacaccataaaaatactcagagatgcgggatatcatgtaaaagcaaatggagtagatgtaacaacacatcgtcaagacattaatggaaaagaaatgaaatttgaagtgttaacattggcaagcttaacaactgaaattcaaatcaacattgagatagaatctagaaaatcctacaaaaaaatgctaaaagaaatgggagaggtagctccagaatacaggcatgactctcctgattgtgggatgataatattatgtatagcagcattagtaataactaaattagcagcaggggacagatctggtcttacagccgtgattaggagagctaataatgtcctaaaaaatgaaatgaaacgttacaaaggcttactacccaaggacatagccaacagcttctatgaagtgtttgaaaaacatccccactttatagatgtttttgttcattttggtatagcacaatcttctaccagaggtggcagtagagttgaagggatttttgcaggattgtttatgaatgcctatggtgcagggcaagtgatgttacggtggggagtcttagcaaaatcggttaaaaatattatgttaggacatgctagtgtgcaagcagaaatggaacaagttgttgaggtttatgaatatgcccaaaaattgggtggtgaagcaggattctaccatatattgaacaacccaaaagcatcattattatctttgactcaatttcctcacttctccagtgtagtattaggcaatgctgctggcctaggcataatgggagagtacagaggtacaccgaggaatcaagatctatatgatgcagcaaaggcatatgctgaacaactcaaagaaaatggtgtgattaactacagtgtactagacttgacagcagaagaactagaggctatcaaacatcagcttaatccaaaagataatgatgtagagctttgagttaataaaaaatggggcaaataaatcatcatggaaaagtttgctcctgaattccatggagaagatgcaaacaacagggctactaaattcctagaatcaataaagggcaaattcacatcacccaaagatcccaagaaaaaagatagtatcatatctgtcaactcaatagatatagaagtaaccaaagaaagccctataacatcaaattcaactattatcaacccaacaaatgagacagatgatactgcagggaacaagcccaattatcaaagaaaacctctagtaagtttcaaagaagaccctacaccaagtgataatcccttttctaaactatacaaagaaaccatagaaacatttgataacaatgaagaagaatccagctattcatacgaagaaataaatgatcagacaaacgataatataacagcaagattagataggattgatgaaaaattaagtgaaatactaggaatgcttcacacattagtagtggcaagtgcaggacctacatctgctcgggatggtataagagatgccatggttggtttaagagaagaaatgatagaaaaaatcagaactgaagcattaatgaccaatgacagattagaagctatggcaagactcaggaatgaggaaagtgaaaagatggcaaaagacacatcagatgaagtgtctctcaatccaacatcagagaaattgaacaacctattggaagggaatgatagtgacaatgatctatcacttgaagatttctgattagttaccaatcttcacatcaacacacaataccaacagaagaccaacaaactaaccaacccaatcatccaaccaaacatccatccgccaatcagccaaacagccaacaaaacaaccagccaatccaaaactaaccacccggaaaaaatctataatatagttacaaaaaaaggaaagggtggggcaaatatggaaacatacgtgaacaagcttcacgaaggctccacatacacagctgctgttcaatacaatgtcttagaaaaagacgatgaccctgcatcacttacaatatgggtgcccatgttccaatcatctatgccagcagatttacttataaaagaactagctaatgtcaacatactagtgaaacaaatatccacacccaagggaccttcactaagagtcatgataaactcaagaagtgcagtgctagcacaaatgcccagcaaatttaccatatgcgctaatgtgtccttggatgaaagaagcaaactagcatatgatgtaaccacaccctgtgaaatcaaggcatgtagtctaacatgcctaaaatcaaaaaatatgttgactacagttaaagatctcactatgaagacactcaaccctacacatgatattattgctttatgtgaatttgaaaacatagtaacatcaaaaaaagtcataataccaacatacctaagatccatcagtgtcagaaataaagatctgaacacacttgaaaatataacaaccactgaattcaaaaatgctatcacaaatgcaaaaatcatcccttactcaggattactattagtcatcacagtgactgacaacaaaggagcattcaaatacataaagccacaaagtcaattcatagtagatcttggagcttacctagaaaaagaaagtatatattatgttaccacaaattggaagcacacagctacacgatttgcaatcaaacccatggaagattaacctttttcctctacatcagtgtgttaattcatacaaactttctacctacattcttcacttcaccatcacaatcacaaacactctgtggttcaaccaatcaaacaaaacttatctgaagtcccagatcatcccaagtcattgtttatcagatctagtactcaaataagttaataaaaaatatacacatggggcaaataatcattggaggaaatccaactaatcacaatatctgttaacatagacaagtccacacaccatacagaatcaaccaatggaaaatacatccataacaatagaattctcaagcaaattctggccttactttacactaatacacatgatcacaacaataatctctttgctaatcataatctccatcatgattgcaatactaaacaaactttgtgaatataacgtattccataacaaaacctttgagttaccaagagctcgagttaatacttgataaagtagttaattaaaaatagtcataacaatgaactaggatatcaagactaacaataacattggggcaaatgcaaacatgtccaaaaacaaggaccaacgcaccgctaagacattagaaaggacctgggacactctcaatcatttattattcatatcatcgtgcttatataagttaaatcttaaatctgtagcacaaatcacattatccattctggcaatgataatctcaacttcacttataattgcagccatcatattcatagcctcggcaaaccacaaagtcacaccaacaactgcaatcatacaagatgcaacaagccagatcaagaacacaaccccaacatacctcacccagaatcctcagcttggaatcagtccctctaatccgtctgaaattacatcacaaatcaccaccatactagcttcaacaacaccaggagtcaagtcaaccctgcaatccacaacagtcaagaccaaaaacacaacaacaactcaaacacaacccagcaagcccaccacaaaacaacgccaaaacaaaccaccaagcaaacccaataatgattttcactttgaagtgttcaactttgtaccctgcagcatatgcagcaacaatccaacctgctgggctatctgcaaaagaataccaaacaaaaaaccaggaaagaaaaccactaccaagcccacaaaaaaaccaaccctcaagacaaccaaaaaagatcccaaacctcaaaccactaaatcaaaggaagtacccaccaccaagcccacagaagagccaaccatcaacaccaccaaaacaaacatcataactacactactcacctccaacaccacaggaaatccagaactcacaagtcaaatggaaaccttccactcaacttcctccgaaggcaatccaagcccttctcaagtctctacaacatccgagtacccatcacaaccttcatctccacccaacacaccacgccagtagttacttaaaaacatattatcacaaaaggccttgaccaacttaaacagaatcaaaataaactctggggcaaataacaatggagttgctaatcctcaaagcaaatgcaattaccacaatcctcactgcagtcacattttgttttgcttctggtcaaaacatcactgaagaattttatcaatcaacatgcagtgcagttagcaaaggctatcttagtgctctgagaactggttggtataccagtgttataactatagaattaagtaatatcaagaaaaataagtgtaatggaacagatgctaaggtaaaattgataaaacaagaattagataaatataaaaatgctgtaacagaattgcagttgctcatgcaaagcacacaagcaacaaacaatcgagccagaagagaactaccaaggtttatgaattatacactcaacaatgccaaaaaaaccaatgtaacattaagcaagaaaaggaaaagaagatttcttggttttttgttaggtgttggatctgcaatcgccagtggcgttgctgtatctaaggtcctgcacctagaaggggaagtgaacaagatcaaaagtgctctactatccacaaacaaggctgtagtcagcttatcaaatggagttagtgttttaaccagcaaagtgttagacctcaaaaactatatagataaacaattgttacctattgtgaacaagcaaagctgcagcatatcaaatatagaaactgtgatagagttccaacaaaagaacaacagactactagagattaccagggaatttagtgttaatgcaggcgtaactacacctgtaagcacttacatgttaactaatagtgaattattgtcattaatcaatgatatgcctataacaaatgatcagaaaaagttaatgtccaacaatgttcaaatagttagacagcaaagttactctatcatgtccataataaaagaggaagtcttagcatatgtagtacaattaccactatatggtgttatagatacaccctgttggaaactacacacatcccctctatgtacaaccaacacaaaagaagggtccaacatctgtttaacaagaactgacagaggatggtactgtgacaatgcaggatcagtatctttcttcccacaagctgaaacatgtaaagttcaatcaaatcgagtattttgtgacacaatgaacagtttaacattaccaagtgaagtaaatctctgcaatgttgacatattcaaccccaaatatgattgtaaaattatgacttcaaaaacagatgtaagcagctccgttatcacatctctaggagccattgtgtcatgctatggcaaaactaaatgtacagcatccaataaaaatcgtggaatcataaagacattttctaacgggtgcgattatgtatcaaataaaggggtggacactgtgtctgtaggtaacacattatattatgtaaataagcaagaaggtaaaagtctctatgtaaaaggtgaaccaataataaatttctatgacccattagtattcccctctgatgaatttgatgcatcaatatctcaagtcaacgagaagattaaccagagcctagcatttattcgtaaatccgatgaattattacataatgtaaatgctggtaaatccaccacaaatatcatgataactactataattatagtgattatagtaatattgttatcattaattgctgttggactgctcttatactgtaaggccagaagcacaccagtcacactaagcaaagatcaactgagtggtataaataatattgcatttagtaactaaataaaaatagcacctaatcatgttcttacaatggtttactatctgctcatagacaacccatctgtcattggattttcttaaaatctgaacttcatcgaaactctcatctataaaccatctcacttacactatttaagtagattcctagtttatagttatataaaacacaattgcatgccagattaacttaccatctgtaaaaatgaaaactggggcaaatatgtcacgaaggaatccttgcaaatttgaaattcgaggtcattgcttaaatggtaagaggtgtcattttagtcataattattttgaatggccaccccatgcactgcttgtaagacaaaactttatgttaaacagaatacttaagtctatggataaaagtatagataccttatcagaaataagtggagctgcagagttggacagaacagaagagtatgctcttggtgtagttggagtgctagagagttatataggatcaataaacaatataactaaacaatcagcatgtgttgccatgagcaaactcctcactgaactcaatagtgatgatatcaaaaagctgagggacaatgaagagctaaattcacccaagataagagtgtacaatactgtcatatcatatattgaaagcaacaggaaaaacaataaacaaactatccatctgttaaaaagattgccagcagacgtattgaagaaaaccatcaaaaacacattggatatccataagagcataaccatcaacaacccaaaagaatcaactgttagtgatacaaatgaccatgccaaaaataatgatactacctgacaaatatccttgtagtataacttccatactaataacaagtagatgtagagttactatgtataatcaaaagaacacactatatttcaatcaaaacaacccaaataaccatatgtactcaccgaatcaaacattcaatgaaatccattggacctctcaagaattgattgacacaattcaaaattttctacaacatctaggtattattgaggatatatatacaatatatatattagtgtcataacactcaattctaacactcaccacatcgttacattattaattcaaacaattcaagttgtgggacaaaatggatcccattattaatggaaattctgctaacgtatacttaaccgatagttatttaaaaggcgtaatcagttttagcgaatgtaacgcattagggtcatatatctttaacggtccatatcttaaaaacgattatactaatctaatcagtagacagaatccgttaatcgaacatatgaatcttaagaaactgaatatcacacaatctttgatcagtaagtatcataaaggcgaaatcaaactcgaagaacctacatattttcaatcactattaatgacatataagtctatgacatctagcgaacagatcgctactactaatctgttgaagaaaattattagacgagctatagagatatctgacgttaaggtatacgctatactgaataaattggggttaaaagagaaagataagataaaatctaataacggtcaagacgaagataatagtgtaattactacaattattaaagacgatatactatccgcagtgaaggataatcaatcacatcttaaagccgataaaaatcatagtactaaacaaaaagatacaattaaaactacattgttaaagaaattgatgtgttctatgcaacatccacctagttggttaatacattggtttaacttatacactaagttgaacaatatacttacacaatatcgatcaaacgaagtgaaaaatcacggttttacattgatagataatcaaacattaagcggatttcaattcatacttaaccaatacggatgtatagtgtatcataaagaattgaaacgtataaccgttacaacatataatcaattcttaacatggaaagatataagtctatctagattgaacgtatgcttaattacatggatttcgaattgtcttaatacacttaataaatcattagggttaagatgcggatttaataacgttatacttacacaattgttcttatacggagattgtatacttaagttgttccataacgaagggttttatataataaaagaggttgagggatttataatgtcattgatactgaatattaccgaagaggatcaatttagaaaaagattctataatagtatgttaaacaatataactgacgcagctaataaagcgcagaagaatctgttatctagagtatgtcatacattgttagacaaaacagtgagcgataatattataaacggtagatggattatactgttatctaaattcttaaaattgattaagttggcaggtgacaataaccttaataacttaagcgaattgtatttcttattcagaatattcggacatcctatggttgacgaacgacaagctatggacgcagtgaagattaattgtaacgaaactaaattctatctattatctagtctatctatgcttagaggcgcattcatatatagaattataaaagggttcgttaataattataatagatggcctacacttagaaacgctatagtgttaccacttagatggttaacatattataaattgaatacatatcctagtttactcgaattaaccgaacgcgatctgatagtgttaagcggacttagattctatagagagtttagattgcctaagaaagtcgatctcgaaatgataattaacgataaggcaattagtccacctaaaaacttaatatggacaagcttccctagaaattatatgcctagtcatatacaaaattatatcgaacacgaaaaattgaaatttagcgaatccgataagtctagaagagtgttagagtattacttacgcgataataaatttaacgaatgcgatctatataattgcgtagtgaaccaatcatatcttaataatcctaatcacgtagtgagtcttacaggtaaggaaagagagttgagcgtaggtagaatgttcgctatgcaacccggtatgtttagacaagtgcaaatactcgcagaaaagatgatagccgaaaatatactgcaattctttcccgaatcattgactagatacggagatttagaattgcaaaagatactcgaattgaaagcaggtatatctaataagtctaatagatataacgataattataataattatatatctaagtgtagtattattaccgatctatctaaattcaatcaggcatttagatacgaaactagttgtatatgctcagacgtattagacgaattacacggagtgcaatctttgtttagttggttacatttaactatacctcacgttacaattatatgtacatatagacacgcaccaccatatataggcgatcatatagtcgatctgaataacgtagacgaacaatccggattgtatagatatcacatgggtggcatagagggatggtgtcaaaaattgtggactatagaggcaattagtctgttagatctaattagtcttaagggtaagttttcgattaccgcattgattaacggtgataatcaatcaattgatatatctaaaccgatacggttaatggagggacaaacacacgctcaagccgattacttactcgcacttaattcacttaaactgttatacaaagagtacgcaggtatagggcataaacttaagggtacagagacatatataagtagggatatgcaatttatgagtaagactatacaacataacggagtgtattatcccgctagtataaagaaagtgcttagagtcggaccttggattaatactatattagacgattttaaggttagtctcgaatcaatcggatcattgacacaagagttggagtatagaggcgaatctctattatgctcattgatttttagaaacgtatggttatacaatcagattgcattgcaattgaaaaatcacgcactatgtaataataagttgtacttagacatacttaaagtgttaaaacatcttaaaacattctttaatctcgataatatagataccgcattaacattgtatatgaatctacctatgttattcggagggggagatcctaatctattgtatagatcattctatagacgtacacctgatttcttaaccgaagctatagtgcatagcgtattcatactatcatattatactaatcacgatcttaaagataagttgcaggatctatctgacgatagattgaataaattcttaacatgtattataacattcgataaaaatcctaacgctgaattcgttacacttatgagagatccacaagcattaggttcagagagacaggctaaaattactagcgaaattaatagattagccgttaccgaagtgttaagtaccgcacctaataagatattctctaaatccgctcaacattatacaacaaccgaaatagatcttaacgatattatgcaaaatatcgaacctacatatcctcacggattacgcgtagtttacgaatcattaccattctataaagccgaaaagatcgttaacttaattagcggtacaaaatcaattactaatatactcgaaaagactagcgcaattgatttaaccgatatagatagagctaccgaaatgatgcgtaaaaatataacattactgatacgtatactaccattagattgtaatagggataaaagagagatactatctatggagaatctatcaattacagaattgtcaaaatacgttagggaacgatcatggtcactatctaatatcgtaggcgtaactagtcctagtattatgtatactatggatattaagtatacaactagtacaattagtagcggtataataatcgaaaaatataacgttaatagtctaacacgtggtgaaaggggacctacaaaaccttgggtcggatctagtacacaagagaagaaaactatgcccgtatataatagacaggtattgactaagaaacaacgagatcaaatagatctattagctaaactcgattgggtatacgctagtatagataataaagacgaatttatggaagagttgtcaatcggtacattagggttaacatacgaaaaagctaagaaattgttcccacaatatctatcagtgaattatctacatagattgacagtgagtagtagaccatgcgaatttcccgctagtatacccgcatatagaactactaattatcatttcgatactagtccaattaatagaatattaaccgaaaaatacggagacgaagatatagatatcgtattccaaaattgtattagtttcggattgagtcttatgtccgtagtcgaacaatttactaacgtatgtcctaataggattatactgatacctaaattgaacgaaatacatcttatgaaacctcctatttttacaggcgatgtcgatatacacaaattgaaacaggttatacaaaaacaacatatgttcttacccgataagatatcgttaacgcaatacgttgagttgttcttatcaaataaaacacttaaatcaggtagtcacgttaatagtaatctgatactcgcacataaaattagcgattactttcataatacatatatattgagtactaacttagccggacattggatactgattatacaattgatgaaagatagtaagggtatattcgaaaaagattggggtgagggatatataaccgatcatatgtttataaaccttaaggtcttctttaacgcatataaaacttatctattatgttttcataagggatacggtaaggctaaactcgaatgcgatatgaatacatccgatctattatgcgtactcgaattaattgatagtagctattggaaatctatgagtaaggtattcttagagcaaaaggtgatcaagtatatactatctcaagacgctagtttgcatagggttaagggatgtcatagttttaaattatggtttcttaaaagattgaacgtagccgaatttacagtatgtccttgggtcgttaacatagattatcatcctacacatatgaaagctatacttacatatatagatctagtgagaatgggattgattaacatagatagaatacatataaagaataaacataaatttaacgacgaattctatactagtaatctattctatataaattataatttttccgataatacacatctattaactaaacatatacgtatagctaatagcgaactcgaaaataattataataaattgtatcatcctacacccgaaacattagagaatatactcgctaatccgattaaatctaacgataagaaaacacttaacgattattgtataggtaaaaacgttgattcaattatgttaccattactatcaaataagaaattgattaaatctagcgctatgattagaactaattatagtaaacaggatctatataacttattccctatggtcgtaattgatagaattatagatcattccggtaataccgctaaatctaatcaattgtatacaactactagtcatcaaatatcattagtgcataatagtactagtctatattgtatgttaccatggcatcatattaatagattcaatttcgtttttagtagtacagggtgtaaaattagtatagagtatatacttaaagatcttaaaattaaagatcctaattgtattgcattcataggcgaaggcgcaggtaatctgttacttagaacagtagtcgaattgcatcccgatattagatatatatatagatcacttaaagattgtaacgatcatagtctaccaatcgaattccttagattgtataacggtcatataaacatagattacggcgaaaacttaacgatacccgctactgacgctactaataatatacattggtcatacttacatattaaattcgcagaacctataagtctattcgtatgcgacgcagaattatccgttacagtgaattggtctaaaattattatcgaatggtctaaacacgttagaaaatgcaaatattgttctagcgttaataagtgtatgttaatcgttaagtatcacgctcaagacgatatagattttaaattagataatataactatacttaaaacatacgtatgcttaggtagtaagcttaagggtagcgaagtatacttagtgttaacgataggtccagctaatatttttcccgtttttaacgtagtgcaaaacgctaaattgattctatctagaactaaaaattttataatgcctaagaaagctgataaagagtcaattgacgctaatataaaatcattgataccattcttatgttatcctataactaagaaagggattaataccgcactatctaaacttaaatccgtagtgagcggagatatactatcttatagtatagccggtagaaacgaagtttttagtaataaattgattaatcataaacatatgaatatacttaaatggtttaatcacgtacttaattttagatcaaccgaattgaattataatcatctatatatggtcgaatctacatatccatacttatccgaactgttaaactcattgactactaacgaattgaagaaattgattaaaattacaggtagtctgttatacaattttcataacgaataatgaataaagatcttataataaaaattcccatagctatacactaacactgtattcaattatagttattaaaaattaaaaatcatataattttttaaataacttttagtgaactaatcctaaagttatcattttaatcttggaggaataaatttaaaccctaatctaattggtttatatgtgtattaactaaattacgagatattagtttttgacactttttttctcgt

SEQ ID NO: 5 - DNA, 15111 bp, Human respiratory syncytial virus
acgggaaaaaatgcgtacaacaaacttgcataaaccaaaaaaatggggcaaataagaatttgataagtaccacttaaatttaactcccttggttagagatgggcagcaattcattgagtatgataaaagtcagattgcaaaatctattcgataatgacgaagtggcactattaaaaattacatgttataccgataaattgatacatctaactaatgcattagctaaagctgtaatacatacaattaaacttaatggaatagtgtttgtacatgtaattacatctagtgatatatgccctaataataatatcgtagtcaagtctaattttacaacaatgccagtgttacaaaatggcggatatatttgggaaatgatggaattgacacattgctcacaacctaatggtctattagacgataattgcgaaattaaatttagtaagaaattatccgatagtacaatgactaattatatgaatcaattatccgaattgttaggtttcgatcttaatccataaattataattaatatcaactagcaaatcaatgtcactaacaccattagttaatataaaacttaacagaagacaaaaatggggcaaataaatcaattcagccaacccaaccatggacacaacccacaatgataatacaccacaaagactgatgattaccgatatgagaccgttgtcacttgagacaattataactagcctaactagagatataataacacataaatttatatatctgattaatcacgaatgcatcgtgaggaaattggacgaaagacaggccacatttacattcttagtcaattacgaaatgaaactattgcataaggtaggctcaactaagtataagaaatataccgaatataacactaaatacggaacattcccaatgcctatattcataaatcacgacgggtttctcgaatgcataggcataaaacctacaaaacatacacccataatctataaatacgatcttaacccataaatttcaacacaatattcacacaatctaaaacaacaactctatgcataactatactccatagtccagatggagcctgaaaattatagtaatttaaaacttaaggagagatataagatagaagatggggcaaatacaaccatggctcttagcaaagtcaagttgaatgatacattgaataaagatcaattactatctagctcgaaatatactatccaacggtctacaggcgattcaatagatacacctaattacgatgtgcaaaaacatattaataaattgtgtggtatgttattgattaccgaagacgcaaatcataaatttacagggttaatcggtatgttatacgctatgtctagattaggtagggaagatacaattaaaatacttagagacgcaggatatcacgttaaagctaacggagtagacgtaactacacatagacaggatattaacggtaaggaaatgaaattcgaagtgttaacactcgctagcttaactaccgaaatacaaattaatatcgaaatcgaatcacgtaaatcttataagaaaatgcttaaagaaatgggcgaagtcgcacccgaatatagacacgatagtcccgattgtggtatgattatactatgtatagccgcattagtgataactaagttggccgcaggcgatagatccggattaaccgcagtgatacgtagagcgaataacgtacttaaaaacgaaatgaaacggtataagggtctattaccaaaagatatagcgaatagtttttacgaagtattcgaaaaacatccacattttatagacgtttttgtgcatttcggaatcgcacaatctagtactagaggaggatctagggttgagggtatattcgcaggattgtttatgaacgcatacggagcaggtcaagtcatgcttagatggggagtactcgcaaaatccgttaaaaatattatgttaggacacgctagcgtacaagccgaaatggaacaagtcgttgaggtatacgaatacgcacaaaaattaggtggagaagcaggattttatcatatactgaataatcctaaagctagtctattaagcttaacacaatttccacatttttctagcgtagtgttaggtaacgcagctggcctaggcataatgggcgaatataggggtacacctagaaatcaggatctatatgacgcagctaaagcatacgctgaacaattgaaagagaatggagtgataaattattccgtactcgatctaacagccgaagagttggaggcaattaaacatcaattgaatccgaaagataatgacgttgagttgtgagttaataaaaaatggggcaaataaatcatcatggaaaagtttgctcctgaattccatggagaagacgcaaataatagggcaacaaaattcttagagtcaatcaagggtaagtttacaagtccaaaagatccaaagaagaaagatagtataataagcgtaaactcaattgatatcgaggtgacaaaggaatcacctataacatctaatagtacaataataaatcccactaacgaaacagacgataccgcaggcaataaacctaattatcaacggaaacccttagtgtcattcaaagaagatccaacacctagtgataatccctttagtaaattgtataaggaaacaatcgaaacattcgataataacgaagaagaatcatcatactcatacgaagagataaacgatcagactaacgataatataaccgctagactagatagaatagacgaaaaactatctgaaatactaggtatgttacacacactagtagtcgcatctgccggacctacaagtgctagagatgggataagggatgcaatggtagggttaagggaagaaatgatagagaaaattagaaccgaagcattaatgactaacgatagactcgaagcaatggctagacttagaaacgaagaatccgaaaagatggcaaaagatacatctgacgaagtgtcacttaatcctactagcgaaaaattgaataatctattagagggaaacgatagtgataacgatctatcactcgaagatttctgattagttaccaatcttcacatcaacacacaataccaacagaagaccaacaaactaaccaacccaatcatccaaccaaacatccatccgccaatcagccaaacagccaacaaaacaaccagccaatccaaaactaaccacccggaaaaaatctataatatagttacaaaaaaaggaaagggtggggcaaatatggaaacatacgtgaacaagcttcacgaaggatcaacatatacagctgcagtccaatataacgtactcgaaaaagacgacgatcccgctagcctaacaatatgggtcccaatgtttcaatctagtatgcccgctgatctattaatcaaagaactagctaacgttaacatactagtcaaacaaattagtacacctaagggaccctcacttagagtgatgattaatagtagatccgcagtcctagcacaaatgcctagtaagtttacaatatgtgctaacgtaagcttagacgaacgatcaaaactagcatacgatgtgacaacaccatgcgaaatcaaagcatgttcattgacatgtcttaaatcaaagaatatgctaacaacagtcaaagatctaacaatgaaaacacttaatcccacacacgatataatcgcactatgcgaattcgaaaatatagtgactagtaagaaagtgataatccctacataccttagatcaatatccgttagaaataaggatctgaatacactcgaaaatataacaacaaccgaattcaaaaacgctataactaacgctaagataatcccttactccggactattgttagtgataaccgtaaccgataataagggagcattcaaatacataaaaccccaatcccaatttatagtcgatttaggcgcatacttagaaaaagaatcaatctattacgttacaactaattggaaacataccgctactagattcgcaatcaaacctatggaagattaacctttttcctctacatcagtgtgttaattcatacaaactttctacctacattcttcacttcaccatcacaatcacaaacactctgtggttcaaccaatcaaacaaaacttatctgaagtcccagatcatcccaagtcattgtttatcagatctagtactcaaataagttaataaaaaatatacacatggggcaaataatcattggaggaaatccaactaatcacaatatctgttaacatagacaagtccacacaccatacagaatcaaccaatggaaaatacatccataacaatagaattctctagcaaattttggccttactttacactaatacacatgataactacaatcatatccctattaatcataatctcaattatgatcgcaatccttaacaaactatgtgagtataacgtattccataacaaaacattcgaattgccaagagctcgagtgaatacctgataaagtagttaattaaaaatagtcataacaatgaactaggatatcaagactaacaataacattggggcaaatgcaaacatgtccaaaaacaaggaccaacgcaccgctaaaacactcgaaaggacatgggatacccttaatcacctattattcataagctcatgcttatataaattgaaccttaaatccgtcgcacagataaccctatcaatactcgcaatgataatctcaacaagcttaatcatagccgcaataatctttatcgctagcgctaaccataaggtaaccccaacaaccgcaattatacaggacgcaacatcccaaatcaaaaacacaaccccaacatacttaacccaaaacccacaactcggaatctcaccctctaacccatccgaaattacctcacagattacaacgatactcgcaagtacaacccccggagtcaaatcgacactccaatcgacaaccgtaaagactaagaatacaacaacaacccaaacccaacctagtaagcctacaactaagcaacgccaaaacaaacctccctctaaaccgaataacgattttcacttcgaagtgttcaatttcgtaccatgctcaatttgctctaataacccaacatgctgggccatatgcaaacgcatcccaaacaagaaacccggaaagaaaacaaccactaagccaacaaagaaaccaacccttaagacaaccaagaaagatccaaaaccccaaacaactaagtctaaagaggtcccaacaactaagccaaccgaagagccaacaatcaatacaactaagactaatataatcacaaccttactgacatctaacacaaccggaaatcccgaactgacatcccaaatggaaacctttcactcaacctctagcgaaggcaatccctcaccatcccaagtctcaaccactagcgaatacccatcccaacctagctcacctcccaatacccctagacagtagttacttaaaaacatattatcacaaaaggccttgaccaacttaaacagaatcaaaataaactctggggcaaataacaatggagttgctaatcctcaaagcaaatgcaatcacaacaatactaacagccgttacattttgtttcgctagcggacaaaacataaccgaagagttttatcaatctacatgttccgccgtaagtaaggggtatctatccgcacttagaaccggatggtatactagcgtaataacaatcgaactatctaatataaagaagaataagtgtaacggtacagacgctaaggttaaattgattaaacaggaactcgataagtataaaaacgccgtaaccgaattgcaattgttaatgcaatctacacaagctactaataatagggctagacgtgaattgcctagatttatgaattatacacttaataacgctaagaaaactaacgttacactatctaagaaacgaaaacgtagattcttagggtttttactcggagtcggttccgcaatcgctagcggagtcgccgtaagtaaagtgttacacctcgaaggcgaagtgaataagataaaatccgcactattatcaactaataaggcagtcgttagcctatctaacggagtcagcgtattgacatctaaagtgttagacttaaagaattatatagataagcaattgttaccaatcgttaataaacaatcatgttcaatatccaatatcgaaaccgtaatcgaatttcaacagaagaataatagattactcgaaattactagagaatttagcgtaaacgctggcgtaacaacacccgtaagtacatatatgttaactaattccgaactgttaagcttaattaacgatatgccaattactaacgatcagaagaaattgatgtctaataacgtacaaatcgttagacagcaatcatattcaattatgtcaattataaaagaagaggtactcgcatacgtagtgcaattacccctatatggcgtaatagatacaccatgttggaaattgcatacaagtccactatgtacaactaatacaaaagagggatctaatatatgcttaactagaaccgatagggggtggtattgcgataacgcaggtagcgtaagtttctttccacaagccgaaacatgtaaagtgcaatctaatagagtgttttgcgatacaatgaatagcttaacactacctagcgaagtcaatctatgtaacgtcgatatattcaatcctaaatatgattgcaaaattatgactagtaagactgacgtaagtagtagcgtaattactagtctcggtgcaatagtgtcatgttatggtaagactaagtgtaccgctagcaataagaatagggggataataaaaacatttagtaacggttgcgattacgttagtaataagggagtcgataccgtaagcgtaggtaatacactatattatgttaataaacaggaaggtaagtcattatacgttaaaggcgaacctataattaatttttacgatccattagtgtttccatccgacgaattcgacgctagtataagtcaggtaaacgaaaagattaaccaatcactcgcattcatacgaaaatccgacgaactgttacacaacgttaacgcaggtaagagtacaactaacataatgataacaacaattataatcgttataatcgttatactgttaagcttaatcgcagtcggattactgttatattgtaaagctagatcaacacccgtaacactatctaaagaccaattatccggtataaataatatcgcattctcaaactaaataaaaatagcacctaatcatgttcttacaatggtttactatctgctcatagacaacccatctgtcattggattttcttaaaatctgaacttcatcgaaactctcatctataaaccatctcacttacactatttaagtagattcctagtttatagttatataaaacacaattgcatgccagattaacttaccatctgtaaaaatgaaaactggggcaaatatgtcacgaaggaatccttgcaaatttgaaattcgaggtcattgcttaaatggtaagaggtgtcattttagtcataattattttgaatggccaccccatgcactgcttgtaagacaaaactttatgttaaacagaatacttaagtctatggataaaagtatagataccttatcagaaataagtggagctgcagagttggacagaacagaagagtatgctcttggtgtagttggagtgctagagagttatataggatcaataaacaatataactaaacaatcagcatgtgttgccatgagcaaactcctcactgaactcaatagtgatgatatcaaaaagctgagggacaatgaagagctaaattcacccaagataagagtgtacaatactgtcatatcatatattgaaagcaacaggaaaaacaataaacaaactatccatctgttaaaaagattgccagcagacgtattgaagaaaaccatcaaaaacacattggatatccataagagcataaccatcaacaacccaaaagaatcaactgttagtgatacaaatgaccatgccaaaaataatgatactacctgacaaatatccttgtagtataacttccatactaataacaagtagatgtagagttactatgtataatcaaaagaacacactatatttcaatcaaaacaacccaaataaccatatgtactcaccgaatcaaacattcaatgaaatccattggacctctcaagaattgattgacacaattcaaaattttctacaacatctaggtattattgaggatatatatacaatatatatattagtgtcataacactcaattctaacactcaccacatcgttacattattaattcaaacaattcaagttgtgggacaaaatggatcccattattaatggaaattctgctaacgtatacttaaccgatagttatttaaaaggcgtaatcagttttagcgaatgtaacgcattagggtcatatatctttaacggtccatatcttaaaaacgattatactaatctaatcagtagacagaatccgttaatcgaacatatgaatcttaagaaactgaatatcacacaatctttgatcagtaagtatcataaaggcgaaatcaaactcgaagaacctacatattttcaatcactattaatgacatataagtctatgacatctagcgaacagatcgctactactaatctgttgaagaaaattattagacgagctatagagatatctgacgttaaggtatacgctatactgaataaattggggttaaaagagaaagataagataaaatctaataacggtcaagacgaagataatagtgtaattactacaattattaaagacgatatactatccgcagtgaaggataatcaatcacatcttaaagccgataaaaatcatagtactaaacaaaaagatacaattaaaactacattgttaaagaaattgatgtgttctatgcaacatccacctagttggttaatacattggtttaacttatacactaagttgaacaatatacttacacaatatcgatcaaacgaagtgaaaaatcacggttttacattgatagataatcaaacattaagcggatttcaattcatacttaaccaatacggatgtatagtgtatcataaagaattgaaacgtataaccgttacaacatataatcaattcttaacatggaaagatataagtctatctagattgaacgtatgcttaattacatggatttcgaattgtcttaatacacttaataaatcattagggttaagatgcggatttaataacgttatacttacacaattgttcttatacggagattgtatacttaagttgttccataacgaagggttttatataataaaagaggttgagggatttataatgtcattgatactgaatattaccgaagaggatcaatttagaaaaagattctataatagtatgttaaacaatataactgacgcagctaataaagcgcagaagaatctgttatctagagtatgtcatacattgttagacaaaacagtgagcgataatattataaacggtagatggattatactgttatctaaattcttaaaattgattaagttggcaggtgacaataaccttaataacttaagcgaattgtatttcttattcagaatattcggacatcctatggttgacgaacgacaagctatggacgcagtgaagattaattgtaacgaaactaaattctatctattatctagtctatctatgcttagaggcgcattcatatatagaattataaaagggttcgttaataattataatagatggcctacacttagaaacgctatagtgttaccacttagatggttaacatattataaattgaatacatatcctagtttactcgaattaaccgaacgcgatctgatagtgttaagcggacttagattctatagagagtttagattgcctaagaaagtcgatctcgaaatgataattaacgataaggcaattagtccacctaaaaacttaatatggacaagcttccctagaaattatatgcctagtcatatacaaaattatatcgaacacgaaaaattgaaatttagcgaatccgataagtctagaagagtgttagagtattacttacgcgataataaatttaacgaatgcgatctatataattgcgtagtgaaccaatcatatcttaataatcctaatcacgtagtgagtcttacaggtaaggaaagagagttgagcgtaggtagaatgttcgctatgcaacccggtatgtttagacaagtgcaaatactcgcagaaaagatgatagccgaaaatatactgcaattctttcccgaatcattgactagatacggagatttagaattgcaaaagatactcgaattgaaagcaggtatatctaataagtctaatagatataacgataattataataattatatatctaagtgtagtattattaccgatctatctaaattcaatcaggcatttagatacgaaactagttgtatatgctcagacgtattagacgaattacacggagtgcaatctttgtttagttggttacatttaactatacctcacgttacaattatatgtacatatagacacgcaccaccatatataggcgatcatatagtcgatctgaataacgtagacgaacaatccggattgtatagatatcacatgggtggcatagagggatggtgtcaaaaattgtggactatagaggcaattagtctgttagatctaattagtcttaagggtaagttttcgattaccgcattgattaacggtgataatcaatcaattgatatatctaaaccgatacggttaatggagggacaaacacacgctcaagccgattacttactcgcacttaattcacttaaactgttatacaaagagtacgcaggtatagggcataaacttaagggtacagagacatatataagtagggatatgcaatttatgagtaagactatacaacataacggagtgtattatcccgctagtataaagaaagtgcttagagtcggaccttggattaatactatattagacgattttaaggttagtctcgaatcaatcggatcattgacacaagagttggagtatagaggcgaatctctattatgctcattgatttttagaaacgtatggttatacaatcagattgcattgcaattgaaaaatcacgcactatgtaataataagttgtacttagacatacttaaagtgttaaaacatcttaaaacattctttaatctcgataatatagataccgcattaacattgtatatgaatctacctatgttattcggagggggagatcctaatctattgtatagatcattctatagacgtacacctgatttcttaaccgaagctatagtgcatagcgtattcatactatcatattatactaatcacgatcttaaagataagttgcaggatctatctgacgatagattgaataaattcttaacatgtattataacattcgataaaaatcctaacgctgaattcgttacacttatgagagatccacaagcattaggttcagagagacaggctaaaattactagcgaaattaatagattagccgttaccgaagtgttaagtaccgcacctaataagatattctctaaatccgctcaacattatacaacaaccgaaatagatcttaacgatattatgcaaaatatcgaacctacatatcctcacggattacgcgtagtttacgaatcattaccattctataaagccgaaaagatcgttaacttaattagcggtacaaaatcaattactaatatactcgaaaagactagcgcaattgatttaaccgatatagatagagctaccgaaatgatgcgtaaaaatataacattactgatacgtatactaccattagattgtaatagggataaaagagagatactatctatggagaatctatcaattacagaattgtcaaaatacgttagggaacgatcatggtcactatctaatatcgtaggcgtaactagtcctagtattatgtatactatggatattaagtatacaactagtacaattagtagcggtataataatcgaaaaatataacgttaatagtctaacacgtggtgaaaggggacctacaaaaccttgggtcggatctagtacacaagagaagaaaactatgcccgtatataatagacaggtattgactaagaaacaacgagatcaaatagatctattagctaaactcgattgggtatacgctagtatagataataaagacgaatttatggaagagttgtcaatcggtacattagggttaacatacgaaaaagctaagaaattgttcccacaatatctatcagtgaattatctacatagattgacagtgagtagtagaccatgcgaatttcccgctagtatacccgcatatagaactactaattatcatttcgatactagtccaattaatagaatattaaccgaaaaatacggagacgaagatatagatatcgtattccaaaattgtattagtttcggattgagtcttatgtccgtagtcgaacaatttactaacgtatgtcctaataggattatactgatacctaaattgaacgaaatacatcttatgaaacctcctatttttacaggcgatgtcgatatacacaaattgaaacaggttatacaaaaacaacatatgttcttacccgataagatatcgttaacgcaatacgttgagttgttcttatcaaataaaacacttaaatcaggtagtcacgttaatagtaatctgatactcgcacataaaattagcgattactttcataatacatatatattgagtactaacttagccggacattggatactgattatacaattgatgaaagatagtaagggtatattcgaaaaagattggggtgagggatatataaccgatcatatgtttataaaccttaaggtcttctttaacgcatataaaacttatctattatgttttcataagggatacggtaaggctaaactcgaatgcgatatgaatacatccgatctattatgcgtactcgaattaattgatagtagctattggaaatctatgagtaaggtattcttagagcaaaaggtgatcaagtatatactatctcaagacgctagtttgcatagggttaagggatgtcatagttttaaattatggtttcttaaaagattgaacgtagccgaatttacagtatgtccttgggtcgttaacatagattatcatcctacacatatgaaagctatacttacatatatagatctagtgagaatgggattgattaacatagatagaatacatataaagaataaacataaatttaacgacgaattctatactagtaatctattctatataaattataatttttccgataatacacatctattaactaaacatatacgtatagctaatagcgaactcgaaaataattataataaattgtatcatcctacacccgaaacattagagaatatactcgctaatccgattaaatctaacgataagaaaacacttaacgattattgtataggtaaaaacgttgattcaattatgttaccattactatcaaataagaaattgattaaatctagcgctatgattagaactaattatagtaaacaggatctatataacttattccctatggtcgtaattgatagaattatagatcattccggtaataccgctaaatctaatcaattgtatacaactactagtcatcaaatatcattagtgcataatagtactagtctatattgtatgttaccatggcatcatattaatagattcaatttcgtttttagtagtacagggtgtaaaattagtatagagtatatacttaaagatcttaaaattaaagatcctaattgtattgcattcataggcgaaggcgcaggtaatctgttacttagaacagtagtcgaattgcatcccgatattagatatatatatagatcacttaaagattgtaacgatcatagtctaccaatcgaattccttagattgtataacggtcatataaacatagattacggcgaaaacttaacgatacccgctactgacgctactaataatatacattggtcatacttacatattaaattcgcagaacctataagtctattcgtatgcgacgcagaattatccgttacagtgaattggtctaaaattattatcgaatggtctaaacacgttagaaaatgcaaatattgttctagcgttaataagtgtatgttaatcgttaagtatcacgctcaagacgatatagattttaaattagataatataactatacttaaaacatacgtatgcttaggtagtaagcttaagggtagcgaagtatacttagtgttaacgataggtccagctaatatttttcccgtttttaacgtagtgcaaaacgctaaattgattctatctagaactaaaaattttataatgcctaagaaagctgataaagagtcaattgacgctaatataaaatcattgataccattcttatgttatcctataactaagaaagggattaataccgcactatctaaacttaaatccgtagtgagcggagatatactatcttatagtatagccggtagaaacgaagtttttagtaataaattgattaatcataaacatatgaatatacttaaatggtttaatcacgtacttaattttagatcaaccgaattgaattataatcatctatatatggtcgaatctacatatccatacttatccgaactgttaaactcattgactactaacgaattgaagaaattgattaaaattacaggtagtctgttatacaattttcataacgaataatgaataaagatcttataataaaaattcccatagctatacactaacactgtattcaattatagttattaaaaattaaaaatcatataattttttaaataacttttagtgaactaatcctaaagttatcattttaatcttggaggaataaatttaaaccctaatctaattggtttatatgtgtattaactaaattacgagatattagtttttgacactttttttctcgt